European Patent Specification EP 3 927 432 B1, published January 28, 2026. Title: ANTIBODIES. Applicant: HARBOUR ANTIBODIES BV et al. The sequence listing filed with the application follows.

SEQUENCE LISTING (655 sequences)

SEQ ID NO: 1 - protein, 98 aa, Homo sapiens
QVQLVESGGGVVQPGRSLRLSCAASGFTFSSYGMHWVRQAPGKGLEWVAVIWYDGSNKYYADSVKGRFTISRDNSKNTLYLQMNSLRAEDTAVYYCAR

SEQ ID NO: 2 - protein, 132 aa, Homo sapiens
QVQLVESGGGVVQPGRSLRLSCTASGFTFSGYGMHWVRQAPGKGLEWVAIIWYDGSNTYYTDSAKGRFTISRDNSKDTLYLQMNSLRVEDTAVYYCARDRGISVAALWKYYYYHGLDVWGQGTTTTVSSAQT

SEQ ID NO: 3 - protein, 132 aa, Homo sapiens
QVQLVESGGGVVQPGRSLRLSCTASGFTFSGYGMHWVRQAPGKGLEWVAIIWYDGSNTYYADSAKGRFTISRDNSKNTLYLQMNSLRVEDTAVYYCARDRGISVAALWKYYYYHGLDVWGQGTTVTVSSAQT

SEQ ID NO: 4 - protein, 132 aa, Homo sapiens
QVQLVESGGGVVQPGMSLRLSCTASGFTFSGYAMHWVRQAPVKGLEWVAIIWYDGSNKYYADSVKGRFTISRDNSKNTLYLQMNSLRAEDTAVYYCARDRGISEAAKWKYYYYYGMDVWGQGTTVTVSSAQT

SEQ ID NO: 5 - protein, 132 aa, Homo sapiens
QVQLVESGGGVVQPGRSLRLSCTASGFTFSGYAMHWVRQAPVKGLEWVAIIWYDGSNKYYADSVKGRFTISRDNSKNTLYLQMNSLRAEDTAVYYCARDRGISEAAKWKYYYYYGMDVWGQGTTVTVSSAQT

SEQ ID NO: 6 - protein, 132 aa, Homo sapiens
QVQLVESGGGVVQTGRSLRLSCAASGFTFSAYAMHWVRQAPGKGLEWVTFIGYEESNKYHADSVKGRFTISRDNSKNTLYLQMNSLRAEDTAVYYCARDRGISVAATWDYYYYYGMDVWGQGTTVTVSSAET

SEQ ID NO: 7 - protein, 131 aa, Homo sapiens
QVQLVESGGGVVQPGRSLRLSCAASGFNFSSDGMHWVRQAPGKGLEWVAVIWYDGRNKYYADSVKGRFTISRDNTKNTLYLQMNSLRAEDTAVYYCARDRGITMGRGPYYYYYGMDVWGQGTTVTVSSAQT

SEQ ID NO: 8 - protein, 131 aa, Homo sapiens
QVQLVESGGGVVQPGRSLRLSCAASGFTFSSDGMHWVRQAPGKGLEWVAVIWYDGSSEYYGDSVKGRFTISRDNSKNTLYLQMNSLRAEDTAVYYCARDRGITMGRGVYYYYYGMDVWGQGTTVTVSSAQT

SEQ ID NO: 9 - protein, 131 aa, Homo sapiens
QVQLVESGGGVVQPGRSLRLSCAASGFTFSSDGMHWVRQAPGKGLEWVAVIWFDGSNKYYADSVKGRFTISRDNSKNTMYLQMNSLRAEDTAVYYCTRDRGITMGRGRYYYYYGMDVWGQGTTVTVSSAQT

SEQ ID NO: 10 - protein, 131 aa, Homo sapiens
QVQLVESGGDVVQPGRSLRLSCAASGITFSNYGMHWVRQAPGKGLEWVAVIWYDGSNKYYADSVKGRFTISRDNSKNTLYLQMNSLRAEDTAVYYCARDRGMTGTTWEYYYYYGMDVWGQGTTVTVSSAQT

SEQ ID NO: 11 - protein, 132 aa, Homo sapiens
QVQLVESGGGVVQPGRSLRLSCAASGFTFSTYAMHWVRQAPGKGLEWVAVIWYDGSNKYYADSVKGRLTISRDNSKNTLFLQMNSLRAEDTAVYYCARDRGITTTDTGYYYYYYGLDIWGQGTTVTVSSAQT

SEQ ID NO: 12 - protein, 132 aa, Homo sapiens
QRKLVESGGGVVQPGRSLRLSCAVSGLIFSNYGMHWVRQAPGKGLEWVAVIWYDGSNTYYTDSVKGRFTISRDNSKNTLYLQMNSLRAEDTAVYYCARDRGMTAPGPGTYYYFYGMDVWGQGTTVTVSSAQT

SEQ ID NO: 13 - protein, 127 aa, Homo sapiens
QVQLVESGGGVVQPGRSLRLSCVASGFTFSNYGMHWVRQTPGKGLEWVAIIWFDGSNKYYADSVKGRFTISRDNSKNTLYLQMNSLRAEDTAVYYCARERGVWNSGWSHAYDIWGQGTMVTVSSAQT

SEQ ID NO: 14 - protein, 127 aa, Homo sapiens; identical to SEQ ID NO: 13

SEQ ID NO: 15 - protein, 130 aa, Homo sapiens
QVQLVESGGGVVQPGRSLRLSCAASGFTFSRYGMHWVRQAPGKGLQWVAFIWYDGSNKYYADAVKVRFTISRDNSKNTLYLQMNSLRAEDTAVYYCATEGDYYGSGSYSRAEYFQEWGQGTLVTVSSAET

SEQ ID NO: 16 - protein, 125 aa, Homo sapiens
QVQLVESGGGVVQPGRSLRLSCAATGFTFSYYGMHWVRQAPGKGLEWVAVIWFDGTNIYYADSVRGRFTISRDNSKNTLYLQMNSLRAEDSAVYYCARDRRSSDWYVVFDYWGQGTLVTVSSAQT

SEQ ID NO: 17 - protein, 125 aa, Homo sapiens
QVQLVESGGGVVQPGRSLRLSCTASGFTFTYYGLHWVRQAPGKGLEWVAVIWYDGSNQYYADSVQGRFTISRDNSKNTLYLQMNSLRAEDTAVYYCAREGLGAVAGYYFDYWGQGTLVTVSAAET

SEQ ID NO: 18 - protein, 120 aa, Homo sapiens
QVQLVESGGGVVQPGRSLRLSCKASGFTFRGYGMHWVRQAPGKGLEWVTVIWHDASNKYYVDSVKGRFSISRDNSKNTLYLQMNSLRAEDTAVYYCARDAGLSFDIWGQGTMVTVSSAQT

SEQ ID NO: 19 - protein, 98 aa, Homo sapiens
QVQLVQSGAEVKKPGSSVKVSCKASGGTFSSYAISWVRQAPGQGLEWMGGIIPIFGTANYAQKFQGRVTITADESTSTAYMELSSLRSEDTAVYYCAR

SEQ ID NO: 20 - protein, 127 aa, Homo sapiens
QVQLVQSGAEVKKPGSSVKISCKASGGTFSTHAFTWVRQAPGQGLEWIGRIIPIFDTPKYAQKFQGRVTIAADISTSTVFMELSSLRSEDTAVFYCAREGYYISGSYRDAFDIWGQGTMVTVSSAQT

SEQ ID NO: 21 - protein, 130 aa, Homo sapiens
QVQLVQSGAEVKKPGSSVKVSCKASGGTFSSYAISWVRQAPGQGLEWMGGIIPIFGTANYAQKFQGRVTITADKSTNTAYMELSSLRSEDTAVYYCAREDITMVRGVITNYWYFDLWGRGTLVTVSSAQT

SEQ ID NO: 22 - protein, 129 aa, Homo sapiens
QVQLVQSGAEVKKPGSSVKVSCKASGGTFSTYAISWVRQAPGQGLEWMGGIIPIFGTANYAQKFQGRVTIIADKSTNTAYMDLSSLRSEDTAVYYCAREGNLGYDVVTGYSYFVYWGQGTLVTVSSAQT

SEQ ID NO: 23 - protein, 127 aa, Homo sapiens
QVQLVQSGAEVKKPGSSVKVSCKASGGTFSSYAISWVRQAPGQGLEWMGGIIPIFGTVKNAQKFQGRVTITADKSTGTAYMELSSLRSEDTAVYYCARDHYYDSNDYYWYFDLWGRGTLVTVSSAQT

SEQ ID NO: 24 - protein, 128 aa, Homo sapiens
QVQLVQSGAEVKKPGSSVKVSCKASGGAFSAYAISWVRQAPGQGLEWMGGIIPIFGTANYAQKFQGRVTITADTSTSTAYMELSSLRSEDTAVYYCAREGDIEVVLAARGFFDYWGQGTLVTVSSAQT

SEQ ID NO: 25 - protein, 128 aa, Homo sapiens
QVQLVQSGTEVKKPGSSVKVSCKASGGAFSAYAITWVRQAPGQGLEWMGGIIPIFGTAHYAQKFQGRVTITADKSTSTAFMELSSLRSEDTAVYYCAREGDIEVVLAGRGYFDYWGQGTLVTVSSAQT

SEQ ID NO: 26 - protein, 128 aa, Homo sapiens
QVQLVQSGAEVKKPGSSVKVSCKASGGAFSAYVITWVRQAPGQGLEWMGGIIPVFGTAHYAQKFQGRVTITADKSTSTAFMELSSLRSEDTAVYYCAREGDIEVVLAGRGYFDYWGQGTLVTVSSAQT

SEQ ID NO: 27 - protein, 128 aa, Homo sapiens
QVQLVQSGAEVKKPGSSVKVSCKASGGAFSAYAIDWVRQAPGQGLEWMGGIIPIFGTAHYAQKLQGRVTITADKSTSTAYMELSSLRSEDTAVYYCAREGDSGLVLAARGFFDYWGQGTLVTVSSAQT

SEQ ID NO: 28 - protein, 128 aa, Homo sapiens
QVQLVQTGAEVKKPGSSVKVSCKASGGTFSIYAISWVRQAPRQGLEWMGGIIPIFGTANYAQKFQGRVTITADKSTNTAYMELSRLRSEDTAVYYCAREGDDVLVPTSRGFFDYWGQGTLVTVSSAQT

SEQ ID NO: 29 - protein, 101 aa, Homo sapiens
QVQLQQSGPGLVKPSQTLSLTCAISGDSVSSNSAAWNWIRQSPSRGLEWLGRTYYRSKWYNDYAVSVKSRITINPDTSKNQFSLQLNSVTPEDTAVYYCAR

SEQ ID NO: 30 - protein, 125 aa, Homo sapiens
QVQLQQSGPGLVKPSQTLSLTCAISGDSVSSNSAAWNWIRQSPSRGLEWLGRTYYRSKWYNDYAVSVKSRITINPNTSKNQFSLQLNPVTPEDTAVYFCAREWFGEGYFDLWGRGTLVTVSSART

SEQ ID NO: 31 - protein, 98 aa, Homo sapiens
QVQLQESGPGLVKPPGTLSLTCAVSGGSISSSNWWSWVRQPPGKGLEWIGEIYHSGSTNYNPSLKSRVTISVDKSKNQFSLKLSSVTAADTAVYCCAR

SEQ ID NO: 32 - protein, 125 aa, Homo sapiens
QVQLQESGPGLVKPSGTLSLTCAVSGGSISSNRWWTWVRRSPGKGLEWIGEIYHSGSTNYNPSLKSRVTISVDRSKNQFSLKLSSVTAADTAVYYCASLTLIWFGEKAFDIWGQGTMVTVSSAET

SEQ ID NO: 33 - protein, 95 aa, Homo sapiens
DIQMTQSPSSLSASVGDRVTITCRASQGISNYLAWYQQKPGKVPKLLIYAASTLQSGVPSRFSGSGSGTDFTLTISSLQPEDVATYYCQKYNSAP

SEQ ID NO: 34 - protein, 113 aa, Homo sapiens
DIQMTQSPSSLSASVGDRVTITCRASQGITNYLAWYQQKPGKVPKLLIYAASILQSGVPSRFSGSGSGTDFTLTISSLQPEDVATFYCQKYNIAPCFFPGRTMEEIKRDDAAP

SEQ ID NO: 35 - protein, 113 aa, Homo sapiens
DIQMTQSPSSLSASVGDRVTITCRASQGITNYLAWYQQKPGKVPQLLIYAASILQSGVPSRFSGSGSGTDFTLTISSLQPEDVATFYCQKYNIVPCFFPGRTMEEIRGDDAAP

SEQ ID NO: 36 - protein, 113 aa, Homo sapiens
DIQMTQSPSSLSASVGDRVTITCRASQDISNYLAWYQQKPGKVPKLLIYAASTLQSGVPSRFSGSGSGTDFTLTISSLQPEDVATYYCQKSNNAPLTFGGGTKVEIKRADAAP

SEQ ID NO: 37 - protein, 113 aa, Homo sapiens
DIQMTQSPSSLSASVGDRVTITCRASQGISNYLAWYQQKPGKVPKLLIYAASTLQSGVPSRFSGSGSGTDFTLTISSLQPEDVATYYCQKYNSAPWTFGQGTKVEIKRADAAP

SEQ ID NO: 38 - protein, 113 aa, Homo sapiens; identical to SEQ ID NO: 37

SEQ ID NO: 39 - protein, 101 aa, Homo sapiens
DIVMTQSPDSLAVSLGERATINCKSSQSVLYSSNNKNYLAWYQQKPGQPPKLLIYWASTRESGVPDRFSGSGSGTDFTLTISSLQAEDVAVYYCQQYYSTP

SEQ ID NO: 40 - protein, 119 aa, Homo sapiens
DIVMTQSPDSLAVSLGERATINCKSSQSVLYGSNNKNYLAWYQQRPGQPPRLLIYWASTRESGVPDRFSGSGPGTDFTLTISSLQAEDVAVYYCQQYYSTPYTFGQGTKLEIKRADAAP

SEQ ID NO: 41 - protein, 94 aa, Homo sapiens
EIVMTQSPATLSVSPGERATLSCRASQSVSSNLAWYQQKPGQAPRLLIYGASTRATGIPARFSGSGSGTEFTLTISSLQSEDFAVYYCQQYNNW

SEQ ID NO: 42 - protein, 113 aa, Homo sapiens
EIVMTQSPATLSVSPGERATLSCRASQSVSSNLTWYQQKPGQAPRLLIYGASTRATGIPTRFSGSGSGTEFTLTISSLQSEDFAVYYCQQYNNWPITFGQGTRLEIKRADAAP

SEQ ID NO: 43 - protein, 113 aa, Homo sapiens; identical to SEQ ID NO: 42

SEQ ID NO: 44 - protein, 113 aa, Homo sapiens
EIVMTQSPATLSVSPGERATLSCRASQSVSSNLAWYQQKPGQAPRLLIYGASTRATGIPARFSGSGSGTEFTLTISSLQSEDFAVYYCQQYNNWPITFGQGTRLEIKRADAAP

SEQ ID NO: 45 - protein, 113 aa, Homo sapiens; identical to SEQ ID NO: 44

SEQ ID NO: 46 - protein, 113 aa, Homo sapiens
EIVMTQSPATLSVSPGERATLSCRAGQSVSSDLAWYQQKPGQAPRLLIYGASTRATGIPARFSGSGSGTEFTLTISSLQSEDFAVYYCQQYNNWPITFGQGTRLEIKRADAAP

SEQ ID NO: 47 - protein, 113 aa, Homo sapiens
EIVMTQSPATLSVSPGERATLSCRASQSVSSNLAWYQQKPGQAPRLLIYGASTRATGIPARFSGSGSGTEFTLTISSLQSEDFAVYYCQQYNNWPLTFGGGTKVEIKRADAAP

SEQ ID NO: 48 - protein, 113 aa, Homo sapiens; identical to SEQ ID NO: 47

SEQ ID NO: 49 - protein, 113 aa, Homo sapiens
EIVMTQSPATLSVSPGERATLSCRASQSVGSNLAWYQQKPGQAPRLLIYGASTRATGIPARFSGSGSGTEFTLTISSLQSEDFAVYYCQQYNNWPLTFGGGTKVEMKRADAAP

SEQ ID NO: 50 - protein, 113 aa, Homo sapiens
EIVMTQSPATLSVSPGERATLSCRASQSVSSNLAWYQQKPGQAPRLLIYGASTRATGIPARFSGSGSGTEFTLTISSLQSEDFAVYYCQQYNNWPYTFGQGTKLEIKRADAAP

SEQ ID NO: 51 - protein, 108 aa, Homo sapiens
EIVMTQSPATLSVSPGERATLSCRASQSVSSNLAWYQQKPGQTPRLLIYGASTRATGVPARFSGSGSGTEFTLTISSLQSEDFAVYYCQQYNNWPLTFGGGTKVEIKR

SEQ ID NO: 52 - protein, 108 aa, Homo sapiens
EIVMTQSPATLSVSPGERATLSCRASQSVSSNLAWYQQKPGQAPRLLIYGASTRATGIPARFSGSGSGTEFTLTISSLQSEDFAVYYCQQYNNWPLTFGGGTKVEIKR

SEQ ID NO: 53 - protein, 108 aa, Homo sapiens
EIVMTQSPATLSVSPGERATLSCRASQSVSINLAWYQQKPGQAPRLLIYDTSARATGIPARFSGSGSGTEFTLTISSLQSEDFAVYYCQQYNNWPFTFGPGTKVDIKR

SEQ ID NO: 54 - protein, 108 aa, Homo sapiens
EIVMTQSPATLSVSPGERATLSCRASQSVSSNLAWYQKKPGQAPRLLIYGASTRVTGIPARFSGSGSGTEFTLTISSLQSEDFAVYYCQQYNNWPLTFGGGTKVEIKR

SEQ ID NO: 55 - protein, 108 aa, Homo sapiens
EIVMTQSPATLSVSPGESATLSCRASQTIYSNLAWYQRKPGQAPRLLIYRASTRATGIPARFSGSGSGTEFTLTISSLQSEDFAVYCCQQFNNWPYTFGQGTKLEIKR

SEQ ID NO: 56 - protein, 108 aa, Homo sapiens
EIVMTQSPATLSVSPGERATLSCGASPSVSTNLAWYQQRPGQAPRLLIYGISTRAAGIPARFSGTGSGTEFTLTISSLQSEDFALYYCQQYNNWPYTFGQGTKLEIKR

SEQ ID NO: 57 - protein, 96 aa, Homo sapiens
EIVLTQSPGTLSLSPGERATLSCRASQSVSSSYLAWYQQKPGQAPRLLIYGASSRATGIPDRFSGSGSGTDFTLTISRLEPEDFAVYYCQQYGSSP

SEQ ID NO: 58 - protein, 107 aa, Homo sapiens
EIVLTQSPGTLSLSPGERATLSCRASQSVSSSYLAWYQQKPGQAPRLLIYGASSRATGIPDRFSGSGSGTDFTLTISRLEPEDFAVYYCQQYGSYTFGQGTKLEIKR

SEQ ID NO: 59 - protein, 108 aa, Homo sapiens
EIVLTQSPGTLSLSPGERATLSCRASQSVSSSYLAWYQQKPDQVPRLLIYGTSSRATGIPDRFSGSGSGTDFTLTISRLEPEDFAVYYCQQYGRSLTFGGGTKVEIKR

SEQ ID NO: 60 - protein, 95 aa, Homo sapiens
DIQLTQSPSFLSASVGDRVTITCRASQGISSYLAWYQQKPGKAPKLLIYAASTLQSGVPSRFSGSGSGTEFTLTISSLQPEDFATYYCQQLNSYP

SEQ ID NO: 61 - protein, 108 aa, Homo sapiens
DIQLTQSPSFLSASVGDRVTITCRASQGISSYLAWYQQKPGKAPKLLIYAASTLQSGVPSRFSGSGSGTEFTLTISSLQPEDFATYYCQQLNSYPWTFGQGTKVEIKR

SEQ ID NO: 62 - protein, 100 aa, Homo sapiens
DIVMTQSPLSLPVTPGEPASISCRSSQSLLHSNGYNYLDWYLQKPGQSPQLLIYLGSNRASGVPDRFSGSGSGTDFTLKISRVEAEDVGVYYCMQALQTP

SEQ ID NO: 63 - protein, 113 aa, Homo sapiens
DIVMTQSPLSLPVTPGEPASISCRSSQSLLHSNGYNYLDWYLQKPGQSPQLLIYLGSNRASGVPDRFSGSGSGTDFTLKISRVEAEDVGIYYCMQALQTPLTFGGGTKVEIKR

SEQ ID NO: 64 - protein, 113 aa, Homo sapiens
DIVMTQSPLSLPVTPGEPASISCRSSQSLLHSNGYNYLDWYLQKPGQSPQLLIYLGSNRASGVPDRFSGSGSGTDFTLKISRVEAEDVGIYYCMQALQTPYTFGQGTKLEIKR

SEQ ID NO: 65 - protein, 113 aa, Homo sapiens; identical to SEQ ID NO: 64

SEQ ID NO: 66 - protein, 95 aa, Homo sapiens
DIQMTQSPSSLSASVGDRVTITCRASQSISSYLNWYQQKPGKAPKLLIYAASSLQSGVPSRFSGSGSGTDFTLTISSLQPEDFATYYCQQSYSTP

SEQ ID NO: 67 - protein, 108 aa, Homo sapiens
DIQMTQSPSSLSASVRDRVTITCRASQIISNYLNWYQQKPGKAPKLLIYAASSLQSGVPSRFSGSGSGTDFTLTISSLQPEDFATYFCQQSYSTPFAFGPGTKVDIKR

SEQ ID NO: 68 - protein, 101 aa, Homo sapiens; identical to SEQ ID NO: 29

SEQ ID NO: 69 - protein, 123 aa, Homo sapiens
QVQLQQSGPGLVKPSQTLSLTCAISGHSVSSNSADWNWIRQSPSRGLEWLGRTYCRSKCYNDYAVSVKSRITINPDTSKNQFSLQLNPVTPEDTAVYYCARSLGSGTYPFDSWGQGTLVTVSS

SEQ ID NO: 70 - protein, 122 aa, Homo sapiens
QVQLQQSGPGLVKPSQTLSLTCAISGDSVSSDSAAWNWIRQSPSRGLEWLGRTYFRSKWNNHYAVSVKSRITINPDTSKNQFSLLLNPVTPEDTAVYYCARATLARGALDYWGQGTLVTVSS

SEQ ID NO: 71 - protein, 95 aa, Homo sapiens; identical to SEQ ID NO: 66

SEQ ID NO: 72 - protein, 108 aa, Homo sapiens
DIQMTQSPSSLSASVGDRVTITCRASQRISRFLNWYQQTPGKAPKFLIYAASSLQSGVPSRFSGSGSGTDFTLTISSLQPEDFATYYCQQSYSTPLTFGGGTTVEIKR

SEQ ID NO: 73 - protein, 101 aa, Homo sapiens; identical to SEQ ID NO: 39

SEQ ID NO: 74 - protein, 114 aa, Homo sapiens
DIVMTQSPDSLAVSLGERATINCKSSQSVLYSSNNMNYLAWYQQKPGQPPKLLIYWASTRESGVPDRFSGSGPGTDFTLTISSLQAEDVAVYYCQQYYSTPWTFGQGTKVEIKR

SEQ ID NO: 75 - protein, 122 aa, Homo sapiens
EVQLVESGGGVVQPGRSLRLSCAASGFTFSSYGMHWVRQAPGKGLEWVAVIWYDGSNKYYADSVKGRFTISRDNSKNTLYLQMNSLRAEDTAVYYCARDERIFGVPDAFDIRGQGTMVTVSS

SEQ ID NO: 76 - protein, 98 aa, Homo sapiens
EVQLVESGGGLVQPGGSLRLSCAASGFTFSSYWMHWVRQAPGKGLVWVSRINSDGSSTSYADSVKGRFTISRDNAKNTLYLQMNSLRAEDTAVYYCAR

SEQ ID NO: 77 - protein, 114 aa, Homo sapiens
EVQLVESGGGLVQPGGSLRLSCAASGFTFSSYWMHWVRQAPGKGLVWVSRINSDGSSTSYADSVKGRFTISRDNAKNTLYLQMNSLRAEDTAVYYCGNPYFDYWGQGTLVTVSS

SEQ ID NO: 78 - protein, 118 aa, Homo sapiens
EVQLVESGGGLVQPGGSLRLSCAASGFTFSSYWMLWVRQAPGEGLVWVSRIDSDGSNTTYADSVKGRFTVSRDNAKNTLYLQMNSLRAEDTAVYYCARSGYGYAFDIWGQGTMVTVSS

SEQ ID NO: 79 - protein, 98 aa, Homo sapiens
EVQLLESGGGLVQPGGSLRLSCAASGFTFSSYAMSWVRQAPGKGLEWVSAISGSGGSTYYADSVKGRFTISRDNSKNTLYLQMNSLRAEDTAVYYCAK

SEQ ID NO: 80 - protein, 120 aa, Homo sapiens
EVQLLESGGGWVQPGGSLRLSCAASGFTFSTNAMSWVRQAPGKGLEWVSGISGSGGSTDYADSVKGRFTISRDNSKNTLYLQMNSLRAEDTAVYYCAPRIAVAPDALDIWGQGTMVTVSS

SEQ ID NO: 81 - protein, 1353 aa, Human betacoronavirus 2c EMC/2012
MIHSVFLLMFLLTPTESYVDVGPDSVKSACIEVDIQQTFFDKTWPRPIDVSKADGIIYPQGRTYSNITITYQGLFPYQGDHGDMYVYSAGHATGTTPQKLFVANYSQDVKQFANGFVVRIGAAANSTGTVIISPSTSATIRKIYPAFMLGSSVGNFSDGKMGRFFNHTLVLLPDGCGTLLRAFYCILEPRSGNHCPAGNSYTSFATYHTPATDCSDGNYNRNASLNSFKEYFNLRNCTFMYTYNITEDEILEWFGITQTAQGVHLFSSRYVDLYGGNMFQFATLPVYDTIKYYSIIPHSIRSIQSDRKAWAAFYVYKLQPLTFLLDFSVDGYIRRAIDCGFNDLSQLHCSYESFDVESGVYSVSSFEAKPSGSVVEQAEGVECDFSPLLSGTPPQVYNFKRLVFTNCNYNLTKLLSLFSVNDFTCSQISPAAIASNCYSSLILDYFSYPLSMKSDLSVSSAGPISQFNYKQSFSNPTCLILATVPHNLTTITKPLKYSYINKCSRLLSDDRTEVPQLVNANQYSPCVSIVPSTVWEDGDYYRKQLSPLEGGGWLVASGSTVAMTEQLQMGFGITVQYGTDTNSVCPKLEFANDTKIASQLGNCVEYSLYGVSGRGVFQNCTAVGVRQQRFVYDAYQNLVGYYSDDGNYYCLRACVSVPVSVIYDKETKTHATLFGSVACEHISSTMSQYSRSTRSMLKRRDSTYGPLQTPVGCVLGLVNSSLFVEDCKLPLGQSLCALPDTPSTLTPRSVRSVPGEMRLASIAFNHPIQVDQLNSSYFKLSIPTNFSFGVTQEYIQTTIQKVTVDCKQYVCNGFQKCEQLLREYGQFCSKINQALHGANLRQDDSVRNLFASVKSSQSSPIIPGFGGDFNLTLLEPVSISTGSRSARSAIEDLLFDKVTIADPGYMQGYDDCMQQGPASARDLICAQYVAGYKVLPPLMDVNMEAAYTSSLLGSIAGVGWTAGLSSFAAIPFAQSIFYRLNGVGITQQVLSENQKLIANKFNQALGAMQTGFTTTNEAFQKVQDAVNNNAQALSKLASELSNTFGAISASIGDIIQRLDVLEQDAQIDRLINGRLTTLNAFVAQQLVRSESAALSAQLAKDKVNECVKAQSKRSGFCGQGTHIVSFVVNAPNGLYFMHVGYYPSNHIEVVSAYGLCDAANPTNCIAPVNGYFIKTNNTRIVDEWSYTGSSFYAPEPITSLNTKYVAPQVTYQNISTNLPPPLLGNSTGIDFQDELDEFFKNVSTSIPNFGSLTQINTTLLDLTYEMLSLQQVVKALNESYIDLKELGNYTYYNKWPWYIWLGFIAGLVALALCVFFILCCTGCGTNCMGKLKCNRCCDRYEEYDLEPHKVHVH

SEQ ID NO: 82 - protein, 13 aa, Human betacoronavirus 2c EMC/2012
DFQDELDEFFKNV

SEQ ID NO: 83 - protein, 10 aa, Homo sapiens
GDSVSSDSAA

SEQ ID NO: 84 - protein, 9 aa, Homo sapiens
TYFRSKWNN

SEQ ID NO: 85 - protein, 12 aa, Homo sapiens
ARATLARGALDY

SEQ ID NO: 86 - protein, 12 aa, Homo sapiens
QSVLYSSNNMNY

SEQ ID NO: 87 - protein, 3 aa, Homo sapiens
WAS

SEQ ID NO: 88 - protein, 9 aa, Homo sapiens
QQYYSTPWT

SEQ ID NO: 89 - protein, 10 aa, Homo sapiens
GHSVSSNSAD

SEQ ID NO: 90 - protein, 9 aa, Homo sapiens
TYCRSKCYN

SEQ ID NO: 91 - protein, 13 aa, Homo sapiens
ARSLGSGTYPFDS

SEQ ID NO: 92 - protein, 6 aa, Homo sapiens
QRISRF

SEQ ID NO: 93 - protein, 3 aa, Homo sapiens
AAS

SEQ ID NO: 94 - protein, 9 aa, Homo sapiens
QQSYSTPLT

SEQ ID NO: 95 - protein, 8 aa, Homo sapiens
GGTFSIYA

SEQ ID NO: 96 - protein, 8 aa, Homo sapiens
IIPIFGTA

SEQ ID NO: 97 - protein, 18 aa, Homo sapiens
AREGDDVLVPTSRGFFDY

SEQ ID NO: 98 - protein, 11 aa, Homo sapiens
QSLLHSNGYNY

SEQ ID NO: 99 - protein, 3 aa, Homo sapiens
LGS

SEQ ID NO: 100 - protein, 9 aa, Homo sapiens
MQALQTPLT

SEQ ID NO: 101 - protein, 8 aa, Homo sapiens
GGAFSAYV

SEQ ID NO: 102 - protein, 8 aa, Homo sapiens
IIPVFGTA

SEQ ID NO: 103 - protein, 18 aa, Homo sapiens
AREGDIEVVLAGRGYFDY

SEQ ID NO: 104 - protein, 11 aa, Homo sapiens
QSLLHSNGYNY

SEQ ID NO: 105 - protein, 3 aa, Homo sapiens
LGS

SEQ ID NO: 106 - protein, 9 aa, Homo sapiens
MQALQTPYT

SEQ ID NO: 107 - protein, 126 aa, Homo sapiens
QVQLVQSGAEVKKPGSSVKVSCKASGGTFSTYAISWVRQAPGQGLEWMGGIIPIFGTANYAQKFQGRVTIIADKSTNTAYMDLSSLRSEDTAVYYCAREGNLGYDVVTGYSYFVYWGQGTLVTVSS

SEQ ID NO: 108 - protein, 108 aa, Homo sapiens; identical to SEQ ID NO: 59

SEQ ID NO: 109 - protein, 8 aa, Homo sapiens
GGTFSTYA

SEQ ID NO: 110 - protein, 8 aa, Homo sapiens
IIPIFGTA

SEQ ID NO: 111 - protein, 19 aa, Homo sapiens
AREGNLGYDVVTGYSYFVY

SEQ ID NO: 112 - protein, 7 aa, Homo sapiens
QSVSSSY

SEQ ID NO: 113 - protein, 3 aa, Homo sapiens
GTS

SEQ ID NO: 114 - protein, 8 aa, Homo sapiens
QQYGRSLT

SEQ ID NO: 115 - protein, 8 aa, Homo sapiens
GFTFSSDG

SEQ ID NO: 116 - protein, 8 aa, Homo sapiens
IWFDGSNK

SEQ ID NO: 117 - protein, 21 aa, Homo sapiens
TRDRGITMGRGRYYYYYGMDV

SEQ ID NO: 118 - protein, 6 aa, Homo sapiens
QSVGSN

SEQ ID NO: 119 - protein, 3 aa, Homo sapiens
GAS

SEQ ID NO: 120 - protein, 9 aa, Homo sapiens
QQYNNWPLT

SEQ ID NO: 121 - protein, 8 aa, Homo sapiens
GGTFSTHA

SEQ ID NO: 122 - protein, 8 aa, Homo sapiens
IIPIFDTP

SEQ ID NO: 123 - protein, 17 aa, Homo sapiens
AREGYYISGSYRDAFDI

SEQ ID NO: 124 - protein, 12 aa, Homo sapiens
QSVLYGSNNKNY

SEQ ID NO: 125 - protein, 3 aa, Homo sapiens
WAS

SEQ ID NO: 126 - protein, 9 aa, Homo sapiens
QQYYSTPYT

SEQ ID NO: 127 - protein, 8 aa, Homo sapiens
GGTFSTYA

SEQ ID NO: 128 - protein, 8 aa, Homo sapiens
IIPIFGTA

SEQ ID NO: 129 - protein, 19 aa, Homo sapiens
AREGNLGYDVVTGYSYFVY

SEQ ID NO: 130 - protein, 7 aa, Homo sapiens
QSVSSSY

SEQ ID NO: 131 - protein, 3 aa, Homo sapiens
GTS

SEQ ID NO: 132 - protein, 8 aa, Homo sapiens
QQYGRSLT

SEQ ID NO: 133 - protein, 9 aa, Homo sapiens
GGSISSNRW

SEQ ID NO: 134 - protein, 7 aa, Homo sapiens
IYHSGST

SEQ ID NO: 135 - protein, 15 aa, Homo sapiens
ASLTLIWFGEKAFDI

SEQ ID NO: 136 - protein, 6 aa, Homo sapiens
PSVSTN

SEQ ID NO: 137 - protein, 3 aa, Homo sapiens
GIS

SEQ ID NO: 138 - protein, 9 aa, Homo sapiens
QQYNNWPYT

SEQ ID NO: 139 - protein, 8 aa, Homo sapiens
GFTFTYYG

SEQ ID NO: 140 - protein, 8 aa, Homo sapiens
IWYDGSNQ

SEQ ID NO: 141 - protein, 15 aa, Homo sapiens
AREGLGAVAGYYFDY

SEQ ID NO: 142 - protein, 6 aa, Homo sapiens
QIISNY

SEQ ID NO: 143 - protein, 3 aa, Homo sapiens
AAS

SEQ ID NO: 144 - protein, 9 aa, Homo sapiens
QQSYSTPFA

SEQ ID NO: 145 - protein, 8 aa, Homo sapiens
GFTFRGYG

SEQ ID NO: 146 - protein, 8 aa, Homo sapiens
IWHDASNK

SEQ ID NO: 147 - protein, 10 aa, Homo sapiens
ARDAGLSFDI

SEQ ID NO: 148 - protein, 7 aa, Homo sapiens
QSVSSSY

SEQ ID NO: 149 - protein, 3 aa, Homo sapiens
GAS

SEQ ID NO: 150 - protein, 7 aa, Homo sapiens
QQYGSYT

SEQ ID NO: 151 - protein, 8 aa, Homo sapiens
GFTFSGYG

SEQ ID NO: 152 - protein, 8 aa, Homo sapiens
IWYDGSNT

SEQ ID NO: 153 - protein, 22 aa, Homo sapiens
ARDRGISVAALWKYYYYHGLDV

SEQ ID NO: 154 - protein, 6 aa, Homo sapiens
QSVSSN

SEQ ID NO: 155 - protein, 3 aa, Homo sapiens
GAS

SEQ ID NO: 156 - protein, 9 aa, Homo sapiens
QQYNNWPIT

SEQ ID NO: 157 - protein, 8 aa, Homo sapiens
GFTFSGYG

SEQ ID NO: 158 - protein, 8 aa, Homo sapiens
IWYDGSNT

SEQ ID NO: 159 - protein, 22 aa, Homo sapiens
ARDRGISVAALWKYYYYHGLDV

SEQ ID NO: 160 - protein, 6 aa, Homo sapiens
QSVSSN

SEQ ID NO: 161 - protein, 3 aa, Homo sapiens
GAS

SEQ ID NO: 162 - protein, 9 aa, Homo sapiens
QQYNNWPIT

SEQ ID NO: 163 - protein, 8 aa, Homo sapiens
GFTFSGYA

SEQ ID NO: 164 - protein, 8 aa, Homo sapiens
IWYDGSNK

SEQ ID NO: 165 - protein, 22 aa, Homo sapiens
ARDRGISEAAKWKYYYYYGMDV

SEQ ID NO: 166 - protein, 6 aa, Homo sapiens
QSVSSN

SEQ ID NO: 167 - protein, 3 aa, Homo sapiens
GAS

SEQ ID NO: 168 - protein, 9 aa, Homo sapiens
QQYNNWPIT

SEQ ID NO: 169 - protein, 8 aa, Homo sapiens
GFTFSGYA

SEQ ID NO: 170 - protein, 8 aa, Homo sapiens
IWYDGSNK

SEQ ID NO: 171 - protein, 22 aa, Homo sapiens
ARDRGISEAAKWKYYYYYGMDV

SEQ ID NO: 172 - protein, 6 aa, Homo sapiens
QSVSSN

SEQ ID NO: 173 - protein, 3 aa, Homo sapiens
GAS

SEQ ID NO: 174 - protein, 9 aa, Homo sapiens
QQYNNWPIT

SEQ ID NO: 175 - protein, 8 aa, Homo sapiens
GFTFSAYA

SEQ ID NO: 176 - protein, 8 aa, Homo sapiens
IGYEESNK

SEQ ID NO: 177 - protein, 22 aa, Homo sapiens
ARDRGISVAATWDYYYYYGMDV

SEQ ID NO: 178 - protein, 6 aa, Homo sapiens
QSVSSD

SEQ ID NO: 179 - protein, 3 aa, Homo sapiens
GAS

SEQ ID NO: 180 - protein, 9 aa, Homo sapiens
QQYNNWPIT

SEQ ID NO: 181 - protein, 8 aa, Homo sapiens
GFNFSSDG

SEQ ID NO: 182 - protein, 8 aa, Homo sapiens
IWYDGRNK

SEQ ID NO: 183 - protein, 21 aa, Homo sapiens
ARDRGITMGRGPYYYYYGMDV

SEQ ID NO: 184 - protein, 6 aa, Homo sapiens
QSVSSN

SEQ ID NO: 185 - protein, 3 aa, Homo sapiens
GAS

SEQ ID NO: 186 - protein, 9 aa, Homo sapiens
QQYNNWPLT

SEQ ID NO: 187 - protein, 8 aa, Homo sapiens
GFTFSSDG

SEQ ID NO: 188 - protein, 8 aa, Homo sapiens
IWYDGSSE

SEQ ID NO: 189 - protein, 21 aa, Homo sapiens
ARDRGITMGRGVYYYYYGMDV

SEQ ID NO: 190 - protein, 6 aa, Homo sapiens
QSVSSN

SEQ ID NO: 191 - protein, 3 aa, Homo sapiens
GAS

SEQ ID NO: 192 - protein, 9 aa, Homo sapiens
QQYNNWPLT

SEQ ID NO: 193 - protein, 8 aa, Homo sapiens
GITFSNYG

SEQ ID NO: 194 - protein, 8 aa, Homo sapiens
IWYDGSNK

SEQ ID NO: 195 - protein, 21 aa, Homo sapiens
ARDRGMTGTTWEYYYYYGMDV

SEQ ID NO: 196 - protein, 6 aa, Homo sapiens
QSVSSN

SEQ ID NO: 197 - protein, 3 aa, Homo sapiens
GAS

SEQ ID NO: 198 - protein, 9 aa, Homo sapiens
QQYNNWPYT

SEQ ID NO: 199 - protein, 8 aa, Homo sapiens
GFTFSTYA

SEQ ID NO: 200 - protein, 8 aa, Homo sapiens
IWYDGSNK

SEQ ID NO: 201 - protein, 22 aa, Homo sapiens
ARDRGITTTDTGYYYYYYGLDI

SEQ ID NO: 202 - protein, 6 aa, Homo sapiens
QSVSSN

SEQ ID NO: 203 - protein, 3 aa, Homo sapiens
GAS

SEQ ID NO: 204 - protein, 9 aa, Homo sapiens
QQYNNWPLT

SEQ ID NO: 205 - protein, 8 aa, Homo sapiens
GLIFSNYG

SEQ ID NO: 206 - protein, 8 aa, Homo sapiens
IWYDGSNT

SEQ ID NO: 207 - protein, 22 aa, Homo sapiens
ARDRGMTAPGPGTYYYFYGMDV

SEQ ID NO: 208 - protein, 6 aa, Homo sapiens
QSVSSN

SEQ ID NO: 209 - protein, 3 aa, Homo sapiens
GAS

SEQ ID NO: 210 - protein, 9 aa, Homo sapiens
QQYNNWPLT

SEQ ID NO: 211 - protein, 8 aa, Homo sapiens
GFTFSNYG

SEQ ID NO: 212 - protein, 8 aa, Homo sapiens
IWFDGSNK

SEQ ID NO: 213 - protein, 17 aa, Homo sapiens
ARERGVWNSGWSHAYDI

SEQ ID NO: 214 - protein, 6 aa, Homo sapiens
QGITNY

SEQ ID NO: 215 - protein, 3 aa, Homo sapiens
AAS

SEQ ID NO: 216 - protein, 9 aa, Homo sapiens
QKYNIAPCF

SEQ ID NO: 217 - protein, 8 aa, Homo sapiens
GFTFSNYG

SEQ ID NO: 218 - protein, 8 aa, Homo sapiens
IWFDGSNK

SEQ ID NO: 219 - protein, 17 aa, Homo sapiens
ARERGVWNSGWSHAYDI

SEQ ID NO: 220 - protein, 6 aa, Homo sapiens
QGITNY

SEQ ID NO: 221 - protein, 3 aa, Homo sapiens
AAS

SEQ ID NO: 222 - protein, 9 aa, Homo sapiens
QKYNIVPCF

SEQ ID NO: 223 - protein, 8 aa, Homo sapiens
GFTFSRYG

SEQ ID NO: 224 - protein, 8 aa, Homo sapiens
IWYDGSNK

SEQ ID NO: 225 - protein, 20 aa, Homo sapiens
ATEGDYYGSGSYSRAEYFQE

SEQ ID NO: 226 - protein, 6 aa, Homo sapiens
QSVSIN

SEQ ID NO: 227 - protein, 3 aa, Homo sapiens
DTS

SEQ ID NO: 228 - protein, 9 aa, Homo sapiens
QQYNNWPFT

SEQ ID NO: 229 - protein, 8 aa, Homo sapiens
GFTFSYYG

SEQ ID NO: 230 - protein, 8 aa, Homo sapiens
IWFDGTNI

SEQ ID NO: 231 - protein, 15 aa, Homo sapiens
ARDRRSSDWYVVFDY

SEQ ID NO: 232 - protein, 6 aa, Homo sapiens
QGISSY

SEQ ID NO: 233 - protein, 3 aa, Homo sapiens
AAS

SEQ ID NO: 234 - protein, 9 aa, Homo sapiens
QQLNSYPWT

SEQ ID NO: 235 - protein, 8 aa, Homo sapiens
GGTFSSYA

SEQ ID NO: 236 - protein, 8 aa, Homo sapiens
IIPIFGTA

SEQ ID NO: 237 - protein, 20 aa, Homo sapiens
AREDITMVRGVITNYWYFDL

SEQ ID NO: 238 - protein, 6 aa, Homo sapiens
QDISNY

SEQ ID NO: 239 - protein, 3 aa, Homo sapiens
AAS

SEQ ID NO: 240 - protein, 9 aa, Homo sapiens
QKSNNAPLT

SEQ ID NO: 241 - protein, 8 aa, Homo sapiens
GGTFSSYA

SEQ ID NO: 242 - protein, 8 aa, Homo sapiens
IIPIFGTV

SEQ ID NO: 243 - protein, 17 aa, Homo sapiens
ARDHYYDSNDYYWYFDL

SEQ ID NO: 244 - protein, 6 aa, Homo sapiens
QSVSSN

SEQ ID NO: 245 - protein, 3 aa, Homo sapiens
GAS

SEQ ID NO: 246 - protein, 9 aa, Homo sapiens
QQYNNWPLT

SEQ ID NO: 247 - protein, 8 aa, Homo sapiens
GGAFSAYA

SEQ ID NO: 248 - protein, 8 aa, Homo sapiens
IIPIFGTA

SEQ ID NO: 249 - protein, 18 aa, Homo sapiens
AREGDIEVVLAARGFFDY

SEQ ID NO: 250 - protein, 6 aa, Homo sapiens
QGISNY

SEQ ID NO: 251 - protein, 3 aa, Homo sapiens
AAS

SEQ ID NO: 252 - protein, 9 aa, Homo sapiens
QKYNSAPWT

SEQ ID NO: 253 - protein, 8 aa, Homo sapiens
GGAFSAYA

SEQ ID NO: 254 - protein, 8 aa, Homo sapiens
IIPIFGTA

SEQ ID NO: 255 - protein, 18 aa, Homo sapiens
AREGDIEVVLAGRGYFDY

SEQ ID NO: 256 - protein, 11 aa, Homo sapiens
QSLLHSNGYNY

SEQ ID NO: 257 - protein, 3 aa, Homo sapiens
LGS

SEQ ID NO: 258 - protein, 9 aa, Homo sapiens
MQALQTPYT

SEQ ID NO: 259 - protein, 8 aa, Homo sapiens
GGAFSAYA

SEQ ID NO: 260 - protein, 8 aa, Homo sapiens
IIPIFGTA

SEQ ID NO: 261 - protein, 18 aa, Homo sapiens
AREGDSGLVLAARGFFDY

SEQ ID NO: 262 - protein, 6 aa, Homo sapiens
QGISNY

SEQ ID NO: 263 - protein, 3 aa, Homo sapiens
AAS

SEQ ID NO: 264 - protein, 9 aa, Homo sapiens
QKYNSAPWT

SEQ ID NO: 265 - protein, 10 aa, Homo sapiens
GDSVSSNSAA

SEQ ID NO: 266 - protein, 9 aa, Homo sapiens
TYYRSKWYN

SEQ ID NO: 267 - protein, 12 aa, Homo sapiens
AREWFGEGYFDL

SEQ ID NO: 268 - protein, 6 aa, Homo sapiens
QTIYSN

SEQ ID NO: 269 - protein, 3 aa, Homo sapiens
RAS

SEQ ID NO: 270 - protein, 9 aa, Homo sapiens
QQFNNWPYT

SEQ ID NO: 271 - protein, 8 aa, Homo sapiens
GFTFSSYG

SEQ ID NO: 272 - protein, 8 aa, Homo sapiens
IWYDGSNK

SEQ ID NO: 273 - protein, 15 aa, Homo sapiens
ARDERIFGVPDAFDI

SEQ ID NO: 274 - protein, 8 aa, Homo sapiens
GFTFSSYW

SEQ ID NO: 275 - protein, 8 aa, Homo sapiens
IDSDGSNT

SEQ ID NO: 276 - protein, 11 aa, Homo sapiens
ARSGYGYAFDI

SEQ ID NO: 277 - protein, 8 aa, Homo sapiens
GFTFSTNA

SEQ ID NO: 278 - protein, 8 aa, Homo sapiens
ISGSGGST

SEQ ID NO: 279 - protein, 13 aa, Homo sapiens
APRIAVAPDALDI

SEQ ID NO: 280 - protein, 8 aa, Homo sapiens
GFTFSSYW

SEQ ID NO: 281 - protein, 8 aa, Homo sapiens
INSDGSST

SEQ ID NO: 282 - protein, 7 aa, Homo sapiens
GNPYFDY

SEQ ID NO: 283 - protein, 129 aa, Homo sapiens
QVQLVESGGGVVQPGRSLRLSCTASGFTFSGYGMHWVRQAPGKGLEWVAIIWYDGSNTYYADSAKGRFTISRDNSKNTLYLQMNSLRVEDTAVYYCARDRGISVAALWKYYYYHGLDVWGQGTTVTVSS

SEQ ID NO: 284 - protein, 108 aa, Homo sapiens
EIVMTQSPATLSVSPGERATLSCRASQSVSSNLTWYQQKPGQAPRLLIYGASTRATGIPTRFSGSGSGTEFTLTISSLQSEDFAVYYCQQYNNWPITFGQGTRLEIKR

SEQ ID NO: 285 - protein, 8 aa, Homo sapiens
GFTFSGYG

SEQ ID NO: 286 - protein, 8 aa, Homo sapiens
IWYDGSNT

SEQ ID NO: 287 - protein, 22 aa, Homo sapiens
ARDRGISVAALWKYYYYHGLDV

SEQ ID NO: 288 - protein, 6 aa, Homo sapiens
QSVSSN

SEQ ID NO: 289 - protein, 3 aa, Homo sapiens
GAS

SEQ ID NO: 290 - protein, 9 aa, Homo sapiens
QQYNNWPIT

SEQ ID NO: 291 - protein, 129 aa, Homo sapiens
QVQLVESGGGVVQPGMSLRLSCTASGFTFSGYAMHWVRQAPVKGLEWVAIIWYDGSNKYYADSVKGRFTISRDNSKNTLYLQMNSLRAEDTAVYYCARDRGISEAAKWKYYYYYGMDVWGQGTTVTVSS

SEQ ID NO: 292 - protein, 108 aa, Homo sapiens
EIVMTQSPATLSVSPGERATLSCRASQSVSSNLAWYQQKPGQAPRLLIYGASTRATGIPARFSGSGSGTEFTLTISSLQSEDFAVYYCQQYNNWPITFGQGTRLEIKR

SEQ ID NO: 293 - protein, 8 aa, Homo sapiens
GFTFSGYA

SEQ ID NO: 294 - protein, 8 aa, Homo sapiens
IWYDGSNK

SEQ ID NO: 295 - protein, 22 aa, Homo sapiens
ARDRGISEAAKWKYYYYYGMDV

SEQ ID NO: 296 - protein, 6 aa, Homo sapiens
QSVSSN

SEQ ID NO: 297 - protein, 3 aa, Homo sapiens
GAS

SEQ ID NO: 298 - protein, 9 aa, Homo sapiens
QQYNNWPIT

SEQ ID NO: 299 - protein, 122 aa, Homo sapiens
QVQLQESGPGLVKPSGTLSLTCAVSGGSISSSKWWSWVRQSPGKGLEWIGEIYHSGSTNYNPSLKSRVTISVDKSKNQFSLKLSSVTAADTAVYYCASLTLIWFGEKAFDIWGQGTMVTVSS

SEQ ID NO: 300 - protein, 108 aa, Homo sapiens
EIVMTQSPATLSVSPGERATLSCRASPSVSSNLAWYQQRPGQAPRLLIYGTSTRATGIPARFSGSGSGTEFTLTISSLQSEDFAVYYCQQYNNWPYTFGQGTKLEIKR

SEQ ID NO: 301 - protein, 9 aa, Homo sapiens
GGSISSSKW

SEQ ID NO: 302 - protein, 7 aa, Homo sapiens
IYHSGST

SEQ ID NO: 303 - protein, 15 aa, Homo sapiens
ASLTLIWFGEKAFDI

SEQ ID NO: 304 - protein, 6 aa, Homo sapiens
PSVSSN

SEQ ID NO: 305 - protein, 3 aa, Homo sapiens
GTS

SEQ ID NO: 306 - protein, 9 aa, Homo sapiens
QQYNNWPYT

SEQ ID NO: 307 - protein, 121 aa, Homo sapiens
EVQLLESGGGLVQPGGSLRLSCAASGFTFSSYAMSWVRQAPGKGLEWVSAISGSGGNTYYADSVKGRFTISRDNSKNTLDLQMNSLRGEDTAVYYCAKDRHNYGYVPFDYWGQGTLVTVSS

SEQ ID NO: 308 - protein, 109 aa, Homo sapiens
EIVMTQSPATLSVSPGERATLSCRASQSVNSNLVWYQQKPGQAPRLLIYGASTRATGIPARFSGSGSGTEFTLTISSLQSEDFAVYYCQQYNTWPPWTFGQGTKVEIKR

SEQ ID NO: 309 - protein, 8 aa, Homo sapiens
GFTFSSYA

SEQ ID NO: 310 - protein, 8 aa, Homo sapiens
ISGSGGNT

SEQ ID NO: 311 - protein, 14 aa, Homo sapiens
AKDRHNYGYVPFDY

SEQ ID NO: 312 - protein, 6 aa, Homo sapiens
QSVNSN

SEQ ID NO: 313 - protein, 3 aa, Homo sapiens
GAS

SEQ ID NO: 314 - protein, 10 aa, Homo sapiens
QQYNTWPPWT

SEQ ID NO: 315 - protein, 116 aa, Homo sapiens
EVQLLESGGGSVQPGGSLRLSCEASGFTFNTYPMSWVRQAPGKGLEWVSGISGSGDRTFYEDSVKGRFTISRDNSKNTLYLQMHSLRGEDTAVYYCAKDLGGEGYWGQGTLVTVSS

SEQ ID NO: 316 - protein, 113 aa, Homo sapiens
QAVVTQESALTTSPGETVTLTCRSSTGAVTTSNYANWVQKKPDHLFTGLIGGTNNRAPGVPARFSGSLIGDKAALTITGAQTEDEAIYFCALWYSNHSVFGGGTKLTVLGQPK

SEQ ID NO: 317 - protein, 8 aa, Homo sapiens
GFTFNTYP

SEQ ID NO: 318 - protein, 8 aa, Homo sapiens
ISGSGDRT

SEQ ID NO: 319 - protein, 9 aa, Homo sapiens
AKDLGGEGY

SEQ ID NO: 320 - protein, 9 aa, Homo sapiens
TGAVTTSNY

SEQ ID NO: 321 - protein, 3 aa, Homo sapiens
GTN

SEQ ID NO: 322 - protein, 9 aa, Homo sapiens
ALWYSNHSV

SEQ ID NO: 323 - protein, 116 aa, Homo sapiens
EVQLLESGGGLVQPGGSLRLSCEDSGVTFSSNPMSWVRQGPGKGLEWVSGISGSGDRTFYEDSVKGRFTISRDNSKNTLYLQMNSLRAEDTAVYYCAKDLGGEGNWGQGTLVTVSS

SEQ ID NO: 324 - protein, 113 aa, Homo sapiens
QAVVTQESALTTSPGETVTLTCRSSTGAVTISNYANWVQEKPDHSFTGLIGGTNNRAPGVPARFSGSLIGDKAALTITGAQTEDEAIYFCALWYNNQSVFGGGTKLTVLGQPK

SEQ ID NO: 325 - protein, 8 aa, Homo sapiens
GVTFSSNP

SEQ ID NO: 326 - protein, 8 aa, Homo sapiens
ISGSGDRT

SEQ ID NO: 327 - protein, 9 aa, Homo sapiens
AKDLGGEGN

SEQ ID NO: 328 - protein, 9 aa, Homo sapiens
TGAVTISNY

SEQ ID NO: 329 - protein, 3 aa, Homo sapiens
GTN

SEQ ID NO: 330 - protein, 9 aa, Homo sapiens
ALWYNNQSV

SEQ ID NO: 331 - protein, 116 aa, Homo sapiens
QVQLVQSGAEVKKPGASVKVSCKASGYTFTSYDINWVRQATGQGLEWMGWMNPISGNTGYAQKFQGRVTMTRNTSRSTAYMELSSLRSEDTAVYYCARGQWLFDYWGQGTLVTVSS

SEQ ID NO: 332 - protein, 108 aa, Homo sapiens
DIQMTQSPSTLSASIGDRVTITCRASQTISSWLAWYQQKPGKAPKLLIYKASSLESGVPSRFSGSGSGTEFTLTISSLQPDDFATYYCQQYNFYSYTFGQGTKLEIRR

SEQ ID NO: 333 - protein, 8 aa, Homo sapiens
GYTFTSYD

SEQ ID NO: 334 - protein, 7 aa, Homo sapiens
MNPISGN

SEQ ID NO: 335 - protein, 9 aa, Homo sapiens
ARGQWLFDY

SEQ ID NO: 336 - protein, 6 aa, Homo sapiens
QTISSW

SEQ ID NO: 337 - protein, 3 aa, Homo sapiens
KAS

SEQ ID NO: 338 - protein, 9 aa, Homo sapiens
QQYNFYSYT

SEQ ID NO: 339 - protein, 126 aa, Homo sapiens
QVQLQQSGPGLVKPSQTLSLTCAISGDSVSSNSAAWNWIRQSPSRGLEWLGRTYYRSKWYNDYAVSVKSRITINPDTSKNQFSLQLNPVTPEDTAVYYCARTITMIRGIIISFDYWGQGTLVTVSS

SEQ ID NO: 340 - protein, 108 aa, Homo sapiens
DIQMTQSPSSLSASVGDRVTITCRASQSISSYLNWYQQKPGKAPKLLIYDASSLQSGVPSRFSGSGSGTDFTLTITSLQPEDFATYYCQQSFITPITFGQGTRLEIKR

SEQ ID NO: 341 - protein, 10 aa, Homo sapiens
GDSVSSNSAA

SEQ ID NO: 342 - protein, 9 aa, Homo sapiens
TYYRSKWYN

SEQ ID NO: 343 - protein, 16 aa, Homo sapiens
ARTITMIRGIIISFDY

SEQ ID NO: 344 - protein, 6 aa, Homo sapiens
QSISSY

SEQ ID NO: 345 - protein, 3 aa, Homo sapiens
DAS

SEQ ID NO: 346 - protein, 9 aa, Homo sapiens
QQSFITPIT

SEQ ID NO: 347 - protein, 122 aa, Homo sapiens
EVQLVESGGGLVQPGRSLRLSCTASGFTFGDYVMSWFRQAPGKGLEWVGFIRSKAHGGTTEYAASVNGRFSISRDDSKTIAYLQMNSLKSEDTAVYYCTWLRNDYYYGMDVWGLGTTVTVSS

SEQ ID NO: 348 - protein, 113 aa, Homo sapiens
DIMMTQSPLSLPVTPGEPASISCRSSQRLLHSNGYSYVDWYLQKPGQSPQLLIYLGSDRASGVPDRFSGSGSGTDFTLKISRVEAEDVGVYYCMQTLQTPWTFGQGTKVEIKR

SEQ ID NO: 349 - protein, 8 aa, Homo sapiens
GFTFGDYV

SEQ ID NO: 350 - protein, 10 aa, Homo sapiens
IRSKAHGGTT

SEQ ID NO: 351 - protein, 13 aa, Homo sapiens
TWLRNDYYYGMDV

SEQ ID NO: 352 - protein, 11 aa, Homo sapiens
QRLLHSNGYSY

SEQ ID NO: 353 - protein, 3 aa, Homo sapiens
LGS

SEQ ID NO: 354 - protein, 9 aa, Homo sapiens
MQTLQTPWT

SEQ ID NO: 355 - protein, 122 aa, Homo sapiens
QVQLVESGGGVVQPGRSLRLSCAASGFTFSKYGMHWVRQAPGKGLEWVANIGYDGSDKYYADSVKGRFTISRDNSKNMLYLQMNSLRAEDTAVYFCARGGWIDDYYYGLDVWGQGTTVTVSS

SEQ ID NO: 356 - protein, 113 aa, Homo sapiens
DIVMTQSPLSLPVIPGEPASISCRSSQSLLHSNGYNYLDWYLQKPGQSPQLLIYLGSNRASGVPDRFSGSGSGTDFSLKISRVEAEDVGVYYCMQVLQTPWTFGQGTKVEIKR

SEQ ID NO: 357 - protein, 8 aa, Homo sapiens
GFTFSKYG

SEQ ID NO: 358 - protein, 8 aa, Homo sapiens
IGYDGSDK

SEQ ID NO: 359 - protein, 15 aa, Homo sapiens
ARGGWIDDYYYGLDV

SEQ ID NO: 360 - protein, 11 aa, Homo sapiens
QSLLHSNGYNY

SEQ ID NO: 361 - protein, 3 aa, Homo sapiens
LGS

SEQ ID NO: 362 - protein, 9 aa, Homo sapiens
MQVLQTPWT

SEQ ID NO: 363 - protein, 122 aa, Homo sapiens
QVQLVESGGGVVQPGRSLRLSCAASGFTFSSYGMHWVRQAPGKGLEWVAVICYDGSDKYYTDSVRGRFTISRDNSKNTLYLQMNSLRVEDTAMYFCARGGWIDDYYYGMDVWGQGTTVTVSS

SEQ ID NO: 364 - protein, 113 aa, Homo sapiens
DIVMTQSPLSLPVTPGEPASISCRSSQSLLHSNGYNYLDWYLQKPGQSPQLLIFLGSNRASGVPDRFSGSGSGTDFTLKISRVEAEDVGAYYCMQVLQTPWTFGQGTKVEIKR

SEQ ID NO: 365 - protein, 8 aa, Homo sapiens
GFTFSSYG

SEQ ID NO: 366 - protein, 8 aa, Homo sapiens
ICYDGSDK

SEQ ID NO: 367 - protein, 15 aa, Homo sapiens
ARGGWIDDYYYGMDV

SEQ ID NO: 368 - protein, 11 aa, Homo sapiens
QSLLHSNGYNY

SEQ ID NO: 369 - protein, 3 aa, Homo sapiens
LGS

SEQ ID NO: 370 - protein, 9 aa, Homo sapiens
MQVLQTPWT

SEQ ID NO: 371 - protein, 122 aa, Homo sapiens
QVQLVESGGGVVQPGRSLRLSCAASGFTFSRYGMHWVRQAPGKGLEWVAVIGYDGSNKYYADSVKGRFTISRDNSKNTLSLQMNSLRAEDTAVYYCARGGWNDDYYYGLDVWGQGTTVTVSS

SEQ ID NO: 372 - protein, 113 aa, Homo sapiens
DIVMTQSPLSLPVIPGEPASISCRSSQSLLHSNGYNYLDWYLQKPGQSPQLLIYLGSNRASGVPDRFSGSGSGTDFTLKISIVEAEDAGVYYCMQVLQTPWTFGQGTKVEIKR

SEQ ID NO: 373 - protein, 8 aa, Homo sapiens
GFTFSRYG

SEQ ID NO: 374 - protein, 8 aa, Homo sapiens
IGYDGSNK

SEQ ID NO: 375 - protein, 15 aa, Homo sapiens
ARGGWNDDYYYGLDV

SEQ ID NO: 376 - protein, 11 aa, Homo sapiens
QSLLHSNGYNY

SEQ ID NO: 377 - protein, 3 aa, Homo sapiens
LGS

SEQ ID NO: 378 - protein, 9 aa, Homo sapiens
MQVLQTPWT

SEQ ID NO: 379 - protein, 126 aa, Homo sapiens
EVQLVESGGGLVQPGGSLRLSCAASGFTFSNYWMTWVRQAPGKGLEWVANIKEDGSEKYYVDSVKGRFTLSRDNAKNSLYLQMNSLRAEDTAVYYCAKEGALLWFGVLRPRAFDIWGQGTMVTVSS

SEQ ID NO: 380 - protein, 113 aa, Homo sapiens
DIVMTQSPLSLPVTPGEPASISCRSSQSLLHSNGYNYLDWYLQNPGQSPHLLIYLASNRASGVPDRFSGSGSGTDFTLKISRVEAADVGVYYCMQALQTPYTFGQGTKLEIKR

SEQ ID NO: 381 - protein, 8 aa, Homo sapiens
GFTFSNYW

SEQ ID NO: 382 - protein, 8 aa, Homo sapiens
IKEDGSEK

SEQ ID NO: 383 - protein, 19 aa, Homo sapiens
AKEGALLWFGVLRPRAFDI

SEQ ID NO: 384 - protein, 11 aa, Homo sapiens
QSLLHSNGYNY

SEQ ID NO: 385 - protein, 3 aa, Homo sapiens
LAS

SEQ ID NO: 386 - protein, 9 aa, Homo sapiens
MQALQTPYT

SEQ ID NO: 387 - protein, 98 aa, Homo sapiens
QVQLVQSGAEVKKPGASVKVSCKASGYTFTSYDINWVRQATGQGLEWMGWMNPNSGNTGYAQKFQGRVTMTRNTSISTAYMELSSLRSEDTAVYYCAR

SEQ ID NO: 388 - protein, 95 aa, Homo sapiens
DIQMTQSPSTLSASVGDRVTITCRASQSISSWLAWYQQKPGKAPKLLIYDASSLESGVPSRFSGSGSGTEFTLTISSLQPDDFATYYCQQYNSYS

SEQ ID NO: 389 - protein, 100 aa, Homo sapiens
EVQLVESGGGLVQPGRSLRLSCTASGFTFGDYAMSWFRQAPGKGLEWVGFIRSKAYGGTTEYTASVKGRFTISRDGSKSIAYLQMNSLKTEDTAVYYCTR

SEQ ID NO: 390 - protein, 98 aa, Homo sapiens
EVQLVESGGGLVQPGGSLRLSCAASGFTFSSYWMSWVRQAPGKGLEWVANIKQDGSEKYYVDSVKGRFTISRDNAKNSLYLQMNSLRAEDTAVYYCAR

SEQ ID NO: 391-392 - skipped (2 entries)

SEQ ID NO: 393 - protein, 20 aa, Homo sapiens
CAREGDDVLVPTSRGFFDYW

SEQ ID NO: 394 - protein, 11 aa, Homo sapiens [sequence omitted]

SEQ ID NO: 395 - protein, 20 aa, Homo sapiens
CAREGDIEVVLAGRGYFDYW

SEQ ID NO: 396 - protein, 11 aa, Homo sapiens [sequence omitted]

SEQ ID NO: 397 - protein, 21 aa, Homo sapiens
CAREGNLGYDVVTGYSYFVYW

SEQ ID NO: 398 - protein, 10 aa, Homo sapiens [sequence omitted]

SEQ ID NO: 399 - protein, 17 aa, Homo sapiens
CASLTLIWFGEKAFDIW

SEQ ID NO: 400 - protein, 11 aa, Homo sapiens [sequence omitted]

SEQ ID NO: 401 - protein, 17 aa, Homo sapiens
CAREGLGAVAGYYFDYW

SEQ ID NO: 402 - protein, 11 aa, Homo sapiens [sequence omitted]

SEQ ID NO: 403 - protein, 12 aa, Homo sapiens
CARDAGLSFDIW

SEQ ID NO: 404 - protein, 9 aa, Homo sapiens [sequence omitted]

SEQ ID NO: 405 - protein, 14 aa, Homo sapiens
CARATLARGALDYW

SEQ ID NO: 406 - protein, 11 aa, Homo sapiens [sequence omitted]

SEQ ID NO: 407 - protein, 15 aa, Homo sapiens
CARSLGSGTYPFDSW

SEQ ID NO: 408 - protein, 11 aa, Homo sapiens [sequence omitted]

SEQ ID NO: 409 - protein, 98 aa, Homo sapiens; identical to SEQ ID NO: 1

SEQ ID NO: 410 - protein, 127 aa, Homo sapiens
EVQLVESGGGVVQPGRSLRLSCAASGFTFSSYGMHWVRQAPGKGLEWVAVIWSDGSNKYYADSVKGRFTISRDNSKNTLYLQMNSLRAEDTAVYYCARDERIFGVPDAFDIWGQGTMVTVSSVPRDC

SEQ ID NO: 411 - protein, 127 aa, Homo sapiens
EVQLVESGGGVVQPGRSLRLSCAASGFTFSSYGMHWVRQAPGKGLEWVAVIWYDGSNKYYADSVKGRFTISRDNSKNTLYLQMNSLRAEDTAVYYCARDERIFGVPDAFDIWGQGTMVTVSSVPRDC

SEQ ID NO: 412 - protein, 127 aa, Homo sapiens
EVQLVESGGSVVQPGRSLRLSCAASGFTFSSYGMHWVRQAPGKGLEWVAVIWSDGSNKYYADSVKGRFTISRDNSKNTLYLQMNSLRAEDTAVYYCARDERIFGVPDAFDIWGQGTMVTVSSVPRDC

SEQ ID NO: 413 - protein, 127 aa, Homo sapiens
EVQLVESGGGLVQPGGSLRLSCAASGFTFSSYGMHWVRQAPGKGLEWVAVIWSDGSNKYYADSVKGRFTISRDNSKNTLYLQMNSLRAEDTAVYYCARDERIFGVPDAFDIWGQGTMVTVSSVPRDC

SEQ ID NO: 414 - protein, 127 aa, Homo sapiens
EVQLVESGGGVVQPGRSLRLSCAASGFTFSTSGMHWVRQAPGKGLEWVAVIWYDGSNKYYADSVKGRFTISRDNSKNTLYLQMNSLRAEDTAVYYCARDERIFGVPDAFDIWGHGTMVTVSSVPRDC

SEQ ID NO: 415 - protein, 127 aa, Homo sapiens
EVQLVESGGGVVQPGRSLRLSCAASGFTFSSYGMHWVRQAPGKGLEWVAVIWSDGSNKYYADSVKGRFTISRDNSKNTLYLQMNNLRAEDTAVYYCARDERIFGVPDAFDIWGQGTMVTVSSVPRDC

SEQ ID NO: 416 - protein, 127 aa, Homo sapiens
EVQLVESGGGVVQPGRSLRLSCAASGFTFSSYGMHWVRQAPGKGLEWVAVIWSDGSNKYYADSVKGRFTISRDNSKNTLYLQMNSLRAEDTAVYYCVRDERIFGVPDTFDIWGQGTMVTVSSVPRDC

SEQ ID NO: 417 - protein, 127 aa, Homo sapiens
EVQLVESGGGVVQPGRSLRLSCAASGFTFSSYGMHWVRQAPGKGLEWVAVIWYDGSNKYYADSVKGRFTISRDNSKNTLYLQMNSLRAEDTAVYYCARDERIFGVPDTFDIRGQGTMVTVSSVPRDC

SEQ ID NO: 418 - protein, 127 aa, Homo sapiens
EVQLVESGGGVVQPGGSLRLSCAASGFTFSSYGMHWVRQAPGKGLEWVAVIWYDGSNKYYADSVKGRFTISRDNSKNTLYLQMNSLRAEDTAVYYCARDERIFGVPDVFDIRGQGTMVTVSSVPRDC

SEQ ID NO: 419 - protein, 127 aa, Homo sapiens
EVQLVESGGGVVQPGRSLRLSCAASGFTFSSYGMHWVRQAPGKGLEWVAVIWYDGSNKYYADSVKGRFTISRDNSKNTLYLQMNSLRAEDTAVYYCARDERIFGVPDAFDIRGQGTMVTVSSVPRDC

SEQ ID NO: 420 - protein, 123 aa, Homo sapiens
EVQLVESGGGVVQPGRSLRLSCAASGFTFSSYGMHWVRQAPGKGLEWVAVIWYDGSNKYYADSVKGRFTISRDNSKNTLYLQMNSLRAEDTAVYYCARDEAGTTFDYWGQGTLVTVSSVPRDC

SEQ ID NO: 421 - protein, 98 aa, Homo sapiens; identical to SEQ ID NO: 76

SEQ ID NO: 422 - protein, 125 aa, Homo sapiens
EVQLVESGGGLVQPGGSLRLSCEASGFIFSHYWMHWVRQAPGKGLVWVSRINSDGSNTSYADSVKGRFTISRDNARNTLYLQMNSLGAEDTAMYYCARGEVGTSYWLNPWGQGTLVTVSSVPRDC

SEQ ID NO: 423 - protein, 119 aa, Homo sapiens
EVQLVESGGGLVQPGGSLRLSCAASGFTFSSYWMHWVRQAPGKGLVWVSRINSDGSSTSYADSVKGRFTISRDNAKNTLYLQMNSLRAEDTAVYYCGNPYFDYWGQGTLVTVSSVPRDC

SEQ ID NO: 424 - protein, 123 aa, Homo sapiens
EVQLVESGGGLVQPGGSLRLSCAASGFTFSSYWMLWVRQAPGEGLVWVSRIDSDGSNTTYADSVKGRFTVSRDNAQNTLYLQMNSLRAEDTAVYYCARSGYGYAFDIWGQGTMVTVSSVPRDC

SEQ ID NO: 425 - protein, 123 aa, Homo sapiens
EVQLVESGGGLVQPGGSLRLSCAASGFTFSSYWMLWVRQAPGEGLVWVSRIDSDGSNTTYADSVKGRFTVSRDNAKNTLYLQMNSLRAEDTAVYYCARSGYGYAFDIWGQGTMVTVSSVPRDC

SEQ ID NO: 426 - protein, 132 aa, Homo sapiens
EVQLVESGGGLVQPGGSLRLSCAASGFTFSNYWMHWVRQAPGKGLVWVSRINSDGSSTSYADSVKGRFTISRDNAKNTLYLLMNSLRAEDTAVYYCARGRDERKGNYYGSEIYPDYWGQGTLVTVSSVPRDC

SEQ ID NO: 427 - protein, 120 aa, Homo sapiens
EVQLVESGGGLVQPGGSLRLSCAASGFTFSNYWMHWVRQAPGKGLVWVSRINTDGSTTSYADSVKGRFTISRDNAKNTLYLLMNSLRAEDTAVYYCARDQYYYVSGQGTMVTVSSVPRDC

SEQ ID NO: 428 - protein, 120 aa, Homo sapiens
EVQLVESGGGLVQPGGSLRLSCAASGFTFSSYWMHWVRQAPGKGLVWVSRINSDGSSTSYADSVKGRFTISRDNAKNTLYLLMNSLRAEDTAVYYCARDQYYYVSGQGTMVTVSSVPRDC

SEQ ID NO: 429 - protein, 120 aa, Homo sapiens
EVQLVESGGGLVQPGGSLRLSCAASGFTFSSYWMHWVRQAPGKGLVWVSRINSDGSSTSYADSVKGRFTISRDNAKNTLYLLMNSLRAEDTAVYYCARDQYYYISGQGTMVTVSSVPRDC

SEQ ID NO: 430 - protein, 98 aa, Homo sapiens; identical to SEQ ID NO: 79

SEQ ID NO: 431 - protein, 125 aa, Homo sapiens
EVQLLESGGGWVQPGGSLRLSCAASGFTFSTNAMSWVRQAPGKGLEWVSGISGSGGSTDYADSVKGRFTISRDNSKNTLYLQMNSLRAEDTAVYYCAPRIAVAPDALDIWGQGTMVTVSSVPRDC

SEQ ID NO: 432 - protein, 120 aa, Homo sapiens
EVQLLESGGGLVQPGGSLRLSCAASGFTFSSYAMSWVRQAPGKGLEWVSAISGSGGNTYYTDSVKGRFTISRDNSKNTLYLQMNSLRAEDTAVYYCAKDLVGAYRGQGTLVTVSSVPRDC

SEQ ID NO: 433 - protein, 125 aa, Homo sapiens
EVQLLESGGGLVQPGGSLRLSCAASGFTFSSFAMSWVRQAPGKGLEWVSAISGSVNSTYYADSVKGRFTISRDNSKNTLYLQMNSLRAEDTAVYYCAKDWASGNYYKDYWGQGTLVTVSSVPRDC

SEQ ID NO: 434 - protein, 125 aa, Homo sapiens
EVQLLESGGGLVQPGGSLRLSCAASGFTFSSYAMSWVRQAPGKGLEWVSAISGNGGSTYYADSVKGRFTISRDNSKNTLYLQMNSLRAEDTAVYYCAKGEQQLAYYFDYWGQGTLVTVSSVPRDC

SEQ ID NO: 435 - protein, 95 aa, Homo sapiens
EIVMTQSPATLSVSPGERATLSCRASQSVSSNLAWYQQKPGQAPRLLIYGASTRATGIPARFSGSGSGTEFTLTISSLQSEDFAVYYCQQYNNWP

SEQ ID NO: 436 - protein, 108 aa, Homo sapiens
EIVMTQSPATLSVSPGERATLSCRASQSVSSNLAWYQQKPGQAPRLLIYGASTRATGIPARFGGSGSGTEFTLSISSLQSEDFAVYYCQHYNNWPLTFGGGTKVEIKK

SEQ ID NO: 437 - protein, 107 aa, Homo sapiens
EIVMTQSPATLSVSPGERATLSCRASQSVSNNLAWYQQKPGQAPRLLIYGASTRATGIPARFSGSGSGTEFTLTISSLQSEDFAVYYCQQYNNWPFTFGPGTKVDIK

SEQ ID NO: 438 - protein, 107 aa, Homo sapiens
EIVMTQSPATRSVSPGERATLSCRASQTISSYLAWYQQKPGQAPGLLIYGASNRATGIPARFSGSGSGTEFTLTISSLQSEDFVIYYRQQYNNWPLTFGGGTKVEIK

SEQ ID NO: 439 - protein, 107 aa, Homo sapiens
EVVMTQSPATLSVSPGERASLSCRASQTVNSNLAWYQQKPGQTPRLLIYGASTRATGIPARFSGSGSGTEFTLTISRLQSEDFTVYYCQQYNNWPLTFGPGTKVDIK

SEQ ID NO: 440 - protein, 107 aa, Homo sapiens
EIVMTQSPATLSVSPGERATLSCRASQSVSSNLAWYQQKPGQAPRLLIYGASTRATGIPARFSGSGSGTEFTLTISSLQSEDFAVYYCQQYNNWPITFGQGTRLEIK

SEQ ID NO: 441 - protein, 107 aa, Homo sapiens
EIVMTQSPATLSVSPGERATLSCRASQSVSSNLAWYQQKPGQAPRLLIFRASTRATGIPARFSGSGSGTEFTLTISSLQSEDFAVYHCQQYNSWPITFGQGTRLEIK

SEQ ID NO: 442 - protein, 107 aa, Homo sapiens
EIVMTQSPATLSVSPGERATLSCRASQSVSSNFAWYQHKPGQAPRLLIYGASTRVTGIPARFSGSGSGTEFTLTISSLQSEDCAIYYCQQYNNWPFTFGPGTKVDIK

SEQ ID NO: 443 - protein, 106 aa, Homo sapiens
ETVMTQSPATLSVSPGERATLSCRASQSVSSNLAWYQQKPGQAPRLLIYGASTRATGIPARFSGSGSGTEFTLTISSLQSEDFAVYYCQQFNNWITFGQGTRLEIK

SEQ ID NO: 444 - protein, 108 aa, Homo sapiens
EIVMTQSPATLSVSPGERATLSCRASQSISSNLAWYQQKPGQAPRLLIYGASTRATGIPARFSGSGSGTEFTLTISSLQSEDFAIYYCQQYNNWPPYTFGQGTKLEIK

SEQ ID NO: 445 - protein, 107 aa, Homo sapiens
EIVMTQSPATLSVSPGERATLSCRASQSVISSLAWYQQTPGQAPRLLIYGASTRATGIPARFSGSGSGTEFTFTISSLQSEDFAVYYCQQYHYWPFTFGPGTKMDIK

SEQ ID NO: 446 - protein, 107 aa, Homo sapiens
RIVMTQSPATLSVSPGERATLSCRASQSVSSNLAWYQQKPGQVPRLLIYGASTRATGIPARFSGSGSGTEFTLTISSLQSEDFAVYYCQQYNNWPFTFGPGTKVDIK

SEQ ID NO: 447 - protein, 107 aa, Homo sapiens
RIVLTQSPATLSVSPGERATLSCRASQSIRSNLAWYQQKPGQAPRHLIYGASTRATGIPARFSGSGSGTDFTLTISSLQSEDFAIYYCQQYNNWPLTFGQGTRLEIK

SEQ ID NO: 448 - protein, 95 aa, Homo sapiens
EIVLTQSPATLSLSPGERATLSCRASQSVSSYLAWYQQKPGQAPRLLIYDASNRATGIPARFSGSGSGTDFTLTISSLEPEDFAVYYCQQRSNWP

SEQ ID NO: 449 - protein, 104 aa, Homo sapiens
EIVLTQSPATLSLSPGERATLSCRASQSVSSSLAWYQQKPGQAPRLLIYDTSNRATGIPARFSGSGSGTDFTLTISSLEPEDFAVYYCQQRSNTFGQGTKLEIK

SEQ ID NO: 450 - protein, 95 aa, Homo sapiens
DIQMTQSPSTLSASVGDRVTITCRASQSISSWLAWYQQKPGKAPKLLIYKASSLESGVPSRFSGSGSGTEFTLTISSLQPDDFATYYCQQYNSYS

SEQ ID NO: 451 - protein, 108 aa, Homo sapiens
DIQMTQSPSTLSASVGDRATITCRASQSISTWLAWYQQKPGKAPKLLIYKASSLESGVPSRFSGSGSGTEFTLTISRLQPDDFATYYCQQYKTYSPFSFGPGTNVDIE

SEQ ID NO: 452 - skipped

SEQ ID NO: 453 - protein, 108 aa, Homo sapiens
DIQMTQSPSTLSASVGDRVTITCRASQSISSWLAWYQQKPGKAPKLLIYKASSLESGVPSRFSGSGSGTEFTLTISSLQSDDFATYYCQQYKSYSPFSFGPGTKVDIK

SEQ ID NO: 454 - protein, 95 aa, Homo sapiens; identical to SEQ ID NO: 60

SEQ ID NO: 455 - protein, 107 aa, Homo sapiens
DIQLTQSPSFLSASVGDRVTITCRASQGISSYLAWYQQKPGKAPKLLIYAASTLQSGVPSRFSGSGSGTEFTLTISSLQPEDFATYYCQQLNSYPLTFGGGTKVEIK

SEQ ID NO: 456 - protein, 107 aa, Homo sapiens
VIQLTQSPSFLSASVGDRVTITCRASQDISSYLAWYQQKPGKAPKLLIYGASTLQSGVPSRFSGSESGTEFTLTISSLQPEDFATYYCQQLNSYPYTFGQGTKLEIK

SEQ ID NO: 457 - protein, 107 aa, Homo sapiens
DIQLTQSPSFRSASVGDRVTITCRASQDISSYLAWYQQKPGKAPKLLIYGASTLQSGVPSRFSGSESGTEFTLTISSLQPEDFATYYCQQLNSYPYTFGQGTKVEIK

SEQ ID NO: 458 - protein, 107 aa, Homo sapiens
DIQLTQSPSFLSASVGDRVTISCRASQGISSYLAWYQQKPGKGPKLLIYAASTLQSGVPSRFSGSGSGTEFTLTISSLQPEDFATYYCQQLNSYPLTFGGGTKVEIK

SEQ ID NO: 459 - protein, 95 aa, Homo sapiens; identical to SEQ ID NO: 33

SEQ ID NO: 460 - protein, 107 aa, Homo sapiens
DIQMTQSPSSLSASVGDRVTITCRASQGINNYLAWYQQKPGKVPKLLIYAASTLQSGVPSRFSGSGSGTDFTLTISSLQPEDVATYYCQKYYSAPLTFGGGTKVEIK

SEQ ID NO: 461 - protein, 95 aa, Homo sapiens; identical to SEQ ID NO: 66

SEQ ID NO: 462 - protein, 107 aa, Homo sapiens
DIQMTQSPSSLSASVGDRVTITCRASQSLGSYLNWFQQKPGKAPKLLIYGAFSLQSGVPSRFSGSGSGTDFTLTISSLQPEDFAIYYCQQSYTTPLTFGGGTKVEIK

SEQ ID NO: 463 - protein, 100 aa, Homo sapiens; identical to SEQ ID NO: 62

SEQ ID NO: 464 - protein, 112 aa, Homo sapiens
DIVMTQSPLSLPVTPGEPASISCRSSQSLLHSNGYNYLDWYLQKPGQSPQLLIYLGSYRASGVPDRFSGSGSGTDFTLKISRVEAEDVGVYYCMQALQTPWTFGQGTKVEIK

SEQ ID NO: 465 - protein, 112 aa, Homo sapiens
DIVMTQSPLSLPVTPEEPASISCRSSQSLLHNNGYNYLDWYLQKPGQSPQLLIYLGSNRASGVPDRFSGSGSGTDFSLKISRVEAEDVGVYYCMQALQTPWTFGQGTKVEIK

SEQ ID NO: 466 - protein, 112 aa, Homo sapiens
DIVMTQSPLSLPVTPGEPASISCRSSQSLLHGNGYNYLDWYLQKPGQSPQLLIYLGSNRASGVPDRFSGSGSGTDFTLKISRVEAEDVGVYYCMQALQTPFTFGPGTKVDIK

SEQ ID NO: 467 - protein, 101 aa, Homo sapiens; identical to SEQ ID NO: 39

SEQ ID NO: 468 - protein, 113 aa, Homo sapiens
DIVMTQSPDSLAVSLGERATINCKSSQSVLASSNNMNYLAWYQQKPGQPPKLLIYWASIRESGVPDRFSGSGPGTDFTLTISSLQTEDVAVYYCHQYYSIPNTFGQGTKLEIK

SEQ ID NO: 469 - protein, 98 aa, Homo sapiens; identical to SEQ ID NO: 1

SEQ ID NO: 470 - protein, 124 aa, Homo sapiens
QVQLVESGGGVVQPGRSLRLSCAVSGFIFSNYGMHWVRQAPGKGLEWVAVIWYDGSKKFHTDSVKGRFTISRDNSKNTLYLQMNSLRAEDTAVYYCARDQGITMVRGLIILDYWGQGTLVTVSS

SEQ ID NO: 471 - protein, 116 aa, Homo sapiens
QVHLVESGGGVVQPGRSLRLSCAASGFTFSSYGMHWVRQGPGKGLEGVAGIWFDGSHEYYADAVKGRFTISRDNSKNTLYLEMSSLRAGDTGIYYCARGGDILTPWGQGSLVIVSS

SEQ ID NO: 472 - protein, 120 aa, Homo sapiens
QVQLVESGGGVVQPGRSLRLSCAASGFTFSSYGIHWVRQAPGKGLEWVALIWYDENNKYYGDSVKGRFTISRDNSKNTLYLQMNSLRAEDTAVYYCAREGDGSYQGMDVWGQGTTVTVSS

SEQ ID NO: 473 - protein, 124 aa, Homo sapiens
QVQLLESGGGVVQPGRSLRLSCAASGSSFSTDVMHWVRQAPGKGLEWVAVIWYDGSNKYYADSVKGRFTISRDNSKNTLYLQMNSLRAEDTAVYYCAREGVYQTFMYPDAFDIWGQGTMVTVSS

SEQ ID NO: 474 - protein, 124 aa, Homo sapiens
QVQLVESGGGVVQPGRSLRLSCAASGFDFSNYGMHWVRQAPGKGLEWVAVIWYDAVNKYYADSVKGRFTISRDNSKNTLYLQMNSLRAEDTAVYYCARDQTYYYDSSGYFFDYWGQGTLVTVSS

SEQ ID NO: 475 - protein, 118 aa, Homo sapiens
LVQLVDSGGGVVQPGRSLRLSCAASGFTFSSYAMHWVRQAPGKGLEWVAVIWFDGSNKFYADSVKGRFTISRDNSKNTMYLQMHSLGAEDTAEYYCARGGAYGLFDYWGQGTLVTVSS

SEQ ID NO: 476 - protein, 124 aa, Homo sapiens
QVQLLESGGGVVQPGRSLRLACAASGFTFSSYVMHWVRQAPGKGLEWVAVIWHDGSNKYYADSVKGRFTISRDNSKNTLYLQMNSLRAEDTAVYYCAREGMYQPLLYPDAFDIWGQGTMVTVSS

SEQ ID NO: 477 - protein, 131 aa, Homo sapiens
QVHLVESGGGVVQPGRSLRLSCAASGFTFSSYGMHWVRQAPGKGLEWVAVIWYDGFNKYYADSVKGRFTISRDNAKNTLYLQMNSLRAEDTAIYYCARSRISNFDILTGYYHYYYYGMDVWGQGTTVTVSS

SEQ ID NO: 478 - protein, 130 aa, Homo sapiens
QVQLVESGGGVVQPGRSLRLSCAASGFTFSSYGMHWVRQAPGKGLEWVAIIWYDENNKYYADSVKGRFTISRDNSKNTLYLQMNSLRAEDTAVYYCTRERAKYYGSGRRDYYYYYGMDVWGQGTTVTVSS

SEQ ID NO: 479 - protein, 123 aa, Homo sapiens
QVQLVESGGGVVQPGKSLRLSCAASGFTFSNYGMHWVRQAPGKGLEWVSFIWYDGSDKGYADSVKGRFTISRDNSKNTLYLQMNSLRAEDTAVYFCAKTPFASSWYGDYFDYWGQGTLVTVSS

SEQ ID NO: 480 - protein, 121 aa, Homo sapiens
QVYLVESGGGVVQPGGSLRLSCAASGFTFGYYGMHWVRQTPGKGLEWVAVIFYDGSNKYYADSAKGRFTISRDNSKNSLSLQMNSLRVEDTAVYYCARGGSNRYYYVLDAWGQGVSVTVSS

SEQ ID NO: 481 - protein, 130 aa, Homo sapiens; identical to SEQ ID NO: 478

SEQ ID NO: 482 - protein, 124 aa, Homo sapiens
QVHLVESGGGVVQPGRSLRLSCAASGFDFNNYGMHWVRQAPGKGLEWVAVIWYDAVNKYYGDSVKGRFTISRDNSKNTLYLQMNSLRAEDTAVYYCARDQTYYYDSSGYFFDCWGQGTLVTVSS

SEQ ID NO: 483 - protein, 121 aa, Homo sapiens
QVQLVESGGGVVQPGRSLRLSCVASGLTFSTYAMHWVRQAPGKGLEWVAVIWDDGINKNYADSVKGRFTISRDNSKKTLFLQMNSLRSEDTAVYFCARDRIPVPGGLFDYWGQGTLVTVSS

SEQ ID NO: 484 - protein, 98 aa, Homo sapiens; identical to SEQ ID NO: 79

SEQ ID NO: 485 - protein, 124 aa, Homo sapiens
EVQLLESGGGLVQPGGSLRLSCAASGFIFSRYAMSWVRQAPGKGLEWVSGISGSGDNPYYADSMKGRFTISRDNSKNTLFLQMNSLRAEDTAVYYCAKGGLLWFGDLLDPFDYWGQGTLVTVSS

SEQ ID NO: 486 - protein, 122 aa, Homo sapiens
EVKLLESGGGLVQPGGSLRLSCAASGFTFSSYAMNWVRQAPGKGLEWVSVVSGSGDYTYYADFVKGRFTISRDNAKNTLYLQMKSLRAEDTAIYYCARTIVWFGELFPSDYWGQGTLVTVSS

SEQ ID NO: 487 - protein, 112 aa, Homo sapiens
EVQLLESGGGLVQPGGSLRLSCAASGFTFSSYAMNWVRQAPGKGLEWVSVISGSGDYTYYADFVKGRFTISRDNSKNTLYLQMNSLRAEDTAIYYCARTIVWFGELFPSDYW

SEQ ID NO: 488 - protein, 123 aa, Homo sapiens
EVQLLESGGGLVQPGGSLRLSCAASGFTFRSYAMSWVRQAPGKGLEWVSGISGSGGITSYADSVKGRFTISRDNSKNTLYLQMNSLRAEDTAVYYCAREDYYGSGSYWYLDLWGRGTLVTVSS

SEQ ID NO: 489 - protein, 119 aa, Homo sapiens
EVQLLESGGGLVQPGGSLRLSCAASGFTFSIYAMNWVRQAPGKGLEWVSGISGSGNHIHYADSVKGRFTISRENSKSTLYLHMNSLRAEDTAVYYCAKDGGLYWYFDLWGRGTLVTVSS

SEQ ID NO: 490 - protein, 119 aa, Homo sapiens; identical to SEQ ID NO: 489

SEQ ID NO: 491 - protein, 122 aa, Homo sapiens
QVQLQQSGPGLVKPSQTLSLTCAISGDNVFSNSAAWNWIRQSPSRGLEWLGRTYYRSKWNNDYAVSVKGRITINPDTYKNQFSLQLNPVTPEDTAVYFCARVPMNRGGMDVWGQGTTVTVSS

SEQ ID NO: 492 - protein, 100 aa, Homo sapiens
EVQLVESGGGLVKPGGSLRLSCAASGFTFSNAWMSWVRQAPGKGLEWVGRIKSKTDGGTTDYAAPVKGRFTISRDDSKNTLYLQMNSLKTEDTAVYYCTT

SEQ ID NO: 493 - protein, 129 aa, Homo sapiens
EVQLVESGGGLVKPGGSLRLSCSASGFTFSNAWMSWVRQAPGKGLEWVGRIKTKTDGGTTDYAAPVKGRFTISRDDSKNTMYLQMNSLKTEDTALYYCSTPGIAAAGTWYYYWYGMDVWGQGTTVTVSS

SEQ ID NO: 494 - protein, 98 aa, Homo sapiens
QVQLVQSGAEVKKPGSSVKVSCKASGGTFSSYAISWVRQAPGQGLEWMGGIIPIFGTANYAQKFQGRVTITADKSTSTAYMELSSLRSEDTAVYYCAR

SEQ ID NO: 495 - protein, 122 aa, Homo sapiens
QVQLVQSGAEVKKPGSSVKVSCKGSGGTFSSYAISWVRQAPGQGLEWMGGIIPFFGATNYAQKFQGRVTITADKSTSTAYMELSSLRSEDTAVYYCARYNWNDNYYYGMDVWGQGTTVTVSS

SEQ ID NO: 496 - protein, 98 aa, Homo sapiens
QVQLQESGPGLVKPSETLSLTCAVSGYSISSGYYWGWIRQPPGKGLEWIGSIYHSGSTYYNPSLKSRVTISVDTSKNQFSLKLSSVTAADTAVYYCAR

SEQ ID NO: 497 - protein, 122 aa, Homo sapiens
QVQLQESGPGLVKPSETLSLTCDVSGHSIRSGYYWGWIRQSPGKGLIWIGSFFYSGNTYYNPSLKSRVTISVDTSKNQFSLNLSSVTAADTAVYYCAGRGHDSGEYVAFDFWGQGTMITVSS

SEQ ID NO: 498 - protein, 97 aa, Homo sapiens
QVQLQQWGAGLLKPSETLSLTCAVYGGSFSGYYWSWIRQPPGKGLEWIGEINHSGSTNYNPSLKSRVTISVDTSKNQFSLKLSSVTAADTAVYYCAR

SEQ ID NO: 499 - protein, 119 aa, Homo sapiens
QVQLRQWGAGLLQPSETLSLTCAVYGESFSGYFWTWIRQAPGKGLEWIGEVDHVGSTNYKPSLESLITISVDTSKNQFSLKLTSVTAADTAVYFCARTGTVFGTSFDYWGQGTLVTVSS

SEQ ID NO: 500 - protein, 6 aa, Homo sapiens
QSVSSN

SEQ ID NO: 501 - protein, 3 aa, Homo sapiens
GAS

SEQ ID NO: 502 - protein, 10 aa, Homo sapiens
QHYNNWPLTF

SEQ ID NO: 503 - protein, 8 aa, Homo sapiens
GFTFRSYA

SEQ ID NO: 504 - protein, 8 aa, Homo sapiens
ISGSGGIT

SEQ ID NO: 505 - protein, 16 aa, Homo sapiens
AREDYYGSGSYWYLDL

SEQ ID NO: 506 - protein, 6 aa, Homo sapiens
QSVSNN

SEQ ID NO: 507 - protein, 3 aa, Homo sapiens
GAS

SEQ ID NO: 508 - protein, 10 aa, Homo sapiens
QQYNNWPFTF

SEQ ID NO: 509 - protein, 8 aa, Homo sapiens
GFTFSSYA

SEQ ID NO: 510 - protein, 8 aa, Homo sapiens
VSGSGDYT

SEQ ID NO: 511 - protein, 15 aa, Homo sapiens
ARTIVWFGELFPSDY

SEQ ID NO: 512 - protein, 6 aa, Homo sapiens
QTISSY

SEQ ID NO: 513 - protein, 3 aa, Homo sapiens
GAS

SEQ ID NO: 514 - protein, 10 aa, Homo sapiens
QQYNNWPLTF

SEQ ID NO: 515 - protein, 8 aa, Homo sapiens
GESFSGYF

SEQ ID NO: 516 - protein, 7 aa, Homo sapiens
VDHVGST

SEQ ID NO: 517 - protein, 13 aa, Homo sapiens
ARTGTVFGTSFDY

SEQ ID NO: 518 - protein, 6 aa, Homo sapiens
QTVNSN

SEQ ID NO: 519 - protein, 3 aa, Homo sapiens
GAS

SEQ ID NO: 520 - protein, 10 aa, Homo sapiens
QQYNNWPLTF

SEQ ID NO: 521 - protein, 9 aa, Homo sapiens
GHSIRSGYY

SEQ ID NO: 522 - protein, 7 aa, Homo sapiens
FFYSGNT

SEQ ID NO: 523 - protein, 15 aa, Homo sapiens
AGRGHDSGEYVAFDF

SEQ ID NO: 524 - protein, 6 aa, Homo sapiens
QSVSSN

SEQ ID NO: 525 - protein, 3 aa, Homo sapiens
GAS

SEQ ID NO: 526 - protein, 10 aa, Homo sapiens
QQYNNWPITF

SEQ ID NO: 527 - protein, 8 aa, Homo sapiens
GFDFNNYG

SEQ ID NO: 528 - protein, 8 aa, Homo sapiens
IWYDAVNK

SEQ ID NO: 529 - protein, 17 aa, Homo sapiens
ARDQTYYYDSSGYFFDC

SEQ ID NO: 530 - protein, 6 aa, Homo sapiens
QSVSSN

SEQ ID NO: 531 - protein, 3 aa, Homo sapiens
RAS

SEQ ID NO: 532 - protein, 10 aa, Homo sapiens
QQYNSWPITF

SEQ ID NO: 533 - protein, 8 aa, Homo sapiens
GFTFSSYG

SEQ ID NO: 534 - protein, 8 aa, Homo sapiens
IWFDGSHE

SEQ ID NO: 535 - protein, 9 aa, Homo sapiens
ARGGDILTP

SEQ ID NO: 536 - protein, 6 aa, Homo sapiens
QSVSSN

SEQ ID NO: 537 - protein, 3 aa, Homo sapiens
GAS

SEQ ID NO: 538 - protein, 10 aa, Homo sapiens
QQYNNWPFTF

SEQ ID NO: 539 - protein, 8 aa, Homo sapiens
GLTFSTYA

SEQ ID NO: 540 - protein, 8 aa, Homo sapiens
IWDDGINK

SEQ ID NO: 541 - protein, 14 aa, Homo sapiens
ARDRIPVPGGLFDY

SEQ ID NO: 542 - protein, 6 aa, Homo sapiens
QSVSSN

SEQ ID NO: 543 - protein, 3 aa, Homo sapiens
GAS

SEQ ID NO: 544 - protein, 9 aa, Homo sapiens
QQFNNWITF

SEQ ID NO: 545 - protein, 8 aa, Homo sapiens
GFTFSIYA

SEQ ID NO: 546 - protein, 8 aa, Homo sapiens
ISGSGNHI

SEQ ID NO: 547 - protein, 12 aa, Homo sapiens
AKDGGLYWYFDL

SEQ ID NO: 548 - protein, 6 aa, Homo sapiens
QSISSN

SEQ ID NO: 549 - protein, 3 aa, Homo sapiens
GAS

SEQ ID NO: 550 - protein, 11 aa, Homo sapiens
QQYNNWPPYTF

SEQ ID NO: 551 - protein, 8 aa, Homo sapiens
GFTFSNYG

SEQ ID NO: 552 - protein, 8 aa, Homo sapiens
IWYDGSDK

SEQ ID NO: 553 - protein, 16 aa, Homo sapiens
AKTPFASSWYGDYFDY

SEQ ID NO: 554 - protein, 6 aa, Homo sapiens
QSVISS

SEQ ID NO: 555 - protein, 3 aa, Homo sapiens
GAS

SEQ ID NO: 556 - protein, 10 aa, Homo sapiens
QQYHYWPFTF

SEQ ID NO: 557 - protein, 8 aa, Homo sapiens
GFDFSNYG

SEQ ID NO: 558 - protein, 8 aa, Homo sapiens
IWYDAVNK

SEQ ID NO: 559 - protein, 17 aa, Homo sapiens
ARDQTYYYDSSGYFFDY

SEQ ID NO: 560 - protein, 6 aa, Homo sapiens
QSVSSN

SEQ ID NO: 561 - protein, 3 aa, Homo sapiens
GAS

SEQ ID NO: 562 - protein, 10 aa, Homo sapiens
QQYNNWPFTF

SEQ ID NO: 563 - protein, 8 aa, Homo sapiens
GFTFSSYA

SEQ ID NO: 564 - protein, 8 aa, Homo sapiens
ISGSGDYT

SEQ ID NO: 565 - protein, 15 aa, Homo sapiens
ARTIVWFGELFPSDY

SEQ ID NO: 566 - protein, 6 aa, Homo sapiens
QSIRSN

SEQ ID NO: 567 - protein, 3 aa, Homo sapiens
GAS

SEQ ID NO: 568 - protein, 10 aa, Homo sapiens
QQYNNWPLTF

SEQ ID NO: 569 - protein, 8 aa, Homo sapiens
GFTFSSYG

SEQ ID NO: 570 - protein, 8 aa, Homo sapiens
IWYDENNK

SEQ ID NO: 571 - protein, 13 aa, Homo sapiens
AREGDGSYQGMDV

SEQ ID NO: 572 - protein, 6 aa, Homo sapiens
QSVSSS

SEQ ID NO: 573 - protein, 3 aa, Homo sapiens
DTS

SEQ ID NO: 574 - protein, 7 aa, Homo sapiens
QQRSNTF

SEQ ID NO: 575 - protein, 8 aa, Homo sapiens
GFTFSSYG

SEQ ID NO: 576 - protein, 8 aa, Homo sapiens
IWYDGFNK

SEQ ID NO: 577 - protein, 24 aa, Homo sapiens
ARSRISNFDILTGYYHYYYYGMDV

SEQ ID NO: 578 - protein, 6 aa, Homo sapiens
QSISTW

SEQ ID NO: 579 - protein, 3 aa, Homo sapiens
KAS

SEQ ID NO: 580 - protein, 11 aa, Homo sapiens
QQYKTYSPFSF

SEQ ID NO: 581 - protein, 8 aa, Homo sapiens
GSSFSTDV

SEQ ID NO: 582 - protein, 8 aa, Homo sapiens
IWYDGSNK

SEQ ID NO: 583 - protein, 17 aa, Homo sapiens
AREGVYQTFMYPDAFDI

SEQ ID NO: 584-586 - skipped (3 entries)

SEQ ID NO: 587 - protein, 8 aa, Homo sapiens
GFTFSIYA

SEQ ID NO: 588 - protein, 8 aa, Homo sapiens
ISGSGNHI

SEQ ID NO: 589 - protein, 12 aa, Homo sapiens
AKDGGLYWYFDL

SEQ ID NO: 590 - protein, 6 aa, Homo sapiens
QSISSW

SEQ ID NO: 591 - protein, 3 aa, Homo sapiens
KAS

SEQ ID NO: 592 - protein, 11 aa, Homo sapiens
QQYKSYSPFSF

SEQ ID NO: 593 - protein, 8 aa, Homo sapiens
GFTFSSYV

SEQ ID NO: 594 - protein, 8 aa, Homo sapiens
IWHDGSNK

SEQ ID NO: 595 - protein, 17 aa, Homo sapiens
AREGMYQPLLYPDAFDI

SEQ ID NO: 596 - protein, 6 aa, Homo sapiens
QGISSY

SEQ ID NO: 597 - protein, 3 aa, Homo sapiens
AAS

SEQ ID NO: 598 - protein, 10 aa, Homo sapiens
QQLNSYPLTF

SEQ ID NO: 599 - protein, 8 aa, Homo sapiens
GFTFSIYA

SEQ ID NO: 600 - protein, 8 aa, Homo sapiens
ISGSGNHI

SEQ ID NO: 601 - protein, 12 aa, Homo sapiens
AKDGGLYWYFDL

SEQ ID NO: 602 - protein, 6 aa, Homo sapiens
QDISSY

SEQ ID NO: 603 - protein, 3 aa, Homo sapiens
GAS

SEQ ID NO: 604 - protein, 10 aa, Homo sapiens
QQLNSYPYTF

SEQ ID NO: 605 - protein, 8 aa, Homo sapiens
GFTFSSYG

SEQ ID NO: 606 - protein, 8 aa, Homo sapiens
IWYDENNK

SEQ ID NO: 607 - protein, 23 aa, Homo sapiens
TRERAKYYGSGRRDYYYYYGMDV

SEQ ID NO: 608 - protein, 6 aa, Homo sapiens
QDISSY

SEQ ID NO: 609 - protein, 3 aa, Homo sapiens
GAS

SEQ ID NO: 610 - protein, 10 aa, Homo sapiens
QQLNSYPYTF

SEQ ID NO: 611 - protein, 8 aa, Homo sapiens
GFTFSSYG

SEQ ID NO: 612 - protein, 8 aa, Homo sapiens
IWYDENNK

SEQ ID NO: 613 - protein, 23 aa, Homo sapiens
TRERAKYYGSGRRDYYYYYGMDV

SEQ ID NO: 614 - protein, 6 aa, Homo sapiens
QGISSY

SEQ ID NO: 615 - protein, 3 aa, Homo sapiens
AAS

SEQ ID NO: 616 - protein, 10 aa, Homo sapiens
QQLNSYPLTF

SEQ ID NO: 617 - protein, 8 aa, Homo sapiens
GFTFGYYG

SEQ ID NO: 618 - protein, 8 aa, Homo sapiens
IFYDGSNK

SEQ ID NO: 619 - protein, 14 aa, Homo sapiens
ARGGSNRYYYVLDA

SEQ ID NO: 620 - protein, 6 aa, Homo sapiens
QGINNY

SEQ ID NO: 621 - protein, 3 aa, Homo sapiens
AAS

SEQ ID NO: 622 - protein, 10 aa, Homo sapiens
QKYYSAPLTF

SEQ ID NO: 623 - protein, 8 aa, Homo sapiens
GFIFSRYA

SEQ ID NO: 624 - protein, 8 aa, Homo sapiens
ISGSGDNP

SEQ ID NO: 625 - protein, 17 aa, Homo sapiens
AKGGLLWFGDLLDPFDY

SEQ ID NO: 626 - protein, 6 aa, Homo sapiens
QSLGSY

SEQ ID NO: 627 - protein, 3 aa, Homo sapiens
GAF

SEQ ID NO: 628 - protein, 10 aa, Homo sapiens
QQSYTTPLTF

SEQ ID NO: 629 - protein, 8 aa, Homo sapiens
GFIFSNYG

SEQ ID NO: 630 - protein, 8 aa, Homo sapiens
IWYDGSKK

SEQ ID NO: 631 - protein, 17 aa, Homo sapiens
ARDQGITMVRGLIILDY

SEQ ID NO: 632 - protein, 11 aa, Homo sapiens
QSLLHSNGYNY

SEQ ID NO: 633 - protein, 3 aa, Homo sapiens
LGS

SEQ ID NO: 634 - protein, 10 aa, Homo sapiens
MQALQTPWTF

SEQ ID NO: 635 - protein, 8 aa, Homo sapiens
GGTFSSYA

SEQ ID NO: 636 - protein, 8 aa, Homo sapiens
IIPFFGAT

SEQ ID NO: 637 - protein, 15 aa, Homo sapiens
ARYNWNDNYYYGMDV

SEQ ID NO: 638 - protein, 11 aa, Homo sapiens
QSLLHNNGYNY

SEQ ID NO: 639 - protein, 3 aa, Homo sapiens
LGS

SEQ ID NO: 640 - protein, 10 aa, Homo sapiens
MQALQTPWTF

SEQ ID NO: 641 - protein, 8 aa, Homo sapiens
GFTFSSYA

SEQ ID NO: 642 - protein, 8 aa, Homo sapiens
IWFDGSNK

SEQ ID NO: 643 - protein, 11 aa, Homo sapiens
ARGGAYGLFDY

SEQ ID NO: 644 - protein, 11 aa, Homo sapiens
QSLLHGNGYNY

SEQ ID NO: 645 - protein, 3 aa, Homo sapiens
LGS

SEQ ID NO: 646 - protein, 10 aa, Homo sapiens
MQALQTPFTF

SEQ ID NO: 647 - protein, 8 aa, Homo sapiens
GFTFSNAW

SEQ ID NO: 648 - protein, 10 aa, Homo sapiens
IKTKTDGGTT

SEQ ID NO: 649 - protein, 20 aa, Homo sapiens
STPGIAAAGTWYYYWYGMDV

SEQ ID NO: 650 - protein, 12 aa, Homo sapiens
QSVLASSNNMNY

SEQ ID NO: 651 - protein, 3 aa, Homo sapiens
WAS

SEQ ID NO: 652 - protein, 10 aa, Homo sapiens
HQYYSIPNTF

SEQ ID NO: 653 - protein, 10 aa, Homo sapiens
GDNVFSNSAA

SEQ ID NO: 654 - protein, 9 aa, Homo sapiens
TYYRSKWNN

SEQ ID NO: 655 - protein, 12 aa, Homo sapiens
ARVPMNRGGMDV